European Patent Application EP 4 190 902 A1, published June 7, 2023. Title: A RECOMBINANT VACCINIA VIRUS. Applicant: TOKYO METROPOLITAN INSTITUTE OF MEDICAL SCIENCE SHIGA UNIVERSITY OF MEDICAL SCIENCE DIRECTOR-GENERAL, NATIONAL INSTITUTE OF INFECTIOUS DISEASES. The sequence listing filed with the application follows.

SEQUENCE LISTING (13 sequences)

SEQ ID NO: 1 - DNA, 8198 bp, Severe acute respiratory syndrome coronavirus 2 (SARS-CoV-2)
  CDS (97)..(8181)
cctgcaggaaaaattgaaaataaatacaaaggttcttgagggttgtgttaaattgaaagcgagaaataatcataaatatgaccgaaaggtaagatgcgggtttgcggtgtaagtgcagcccgtcttacaccgtgcggcacaggcactagtactgatgtcgtatacagggcttttgacatctacaatgataaagtagctggttttgctaaattcctaaaaactaattgttgtcgcttccaagaaaaggacgaagatgacaatttaattgattcttactttgtagttaagagacacactttctctaactaccaacatgaagaaacaatttataatttacttaaggattgtccagctgttgctaaacatgacttctttaagtttagaatagacggtgacatggtaccacatatatcacgtcaacgtcttactaaatacacaatggcagacctcgtctatgctttaaggcattttgatgaaggtaattgtgacacattaaaagaaatacttgtcacatacaattgttgtgatgatgattatttcaataaaaaggactggtatgattttgtagaaaacccagatatattacgcgtatacgccaacttaggtgaacgtgtacgccaagctttgttaaaaacagtacaattctgtgatgccatgcgaaatgctggtattgttggtgtactgacattagataatcaagatctcaatggtaactggtatgatttcggtgatttcatacaaaccacgccaggtagtggagttcctgttgtagattcttattattcattgttaatgcctatattaaccttgaccagggctttaactgcagagtcacatgttgacactgacttaacaaagccttacattaagtgggatttgttaaaatatgacttcacggaagagaggttaaaactctttgaccgttattttaaatattgggatcagacataccacccaaattgtgttaactgtttggatgacagatgcattctgcattgtgcaaactttaatgttttattctctacagtgttcccacctacaagttttggaccactagtgagaaaaatatttgttgatggtgttccatttgtagtttcaactggataccacttcagagagctaggtgttgtacataatcaggatgtaaacttacatagctctagacttagttttaaggaattacttgtgtatgctgctgaccctgctatgcacgctgcttctggtaatctattactagataaacgcactacgtgcttttcagtagctgcacttactaacaatgttgcttttcaaactgtcaaacccggtaattttaacaaagacttctatgactttgctgtgtctaagggtttctttaaggaaggaagttctgttgaattaaaacacttcttctttgctcaggatggtaatgctgctatcagcgattatgactactatcgttataatctaccaacaatgtgtgatatcagacaactactatttgtagttgaagttgttgataagtactttgattgttacgatggtggctgtattaatgctaaccaagtcatcgtcaacaacctagacaaatcagctggttttccatttaataaatggggtaaggctagactttattatgattcaatgagttatgaggatcaagatgcacttttcgcatatacaaaacgtaatgtcatccctactataactcaaatgaatcttaagtatgccattagtgcaaagaatagagctcgcaccgtagctggtgtctctatctgtagtactatgaccaatagacagtttcatcaaaaattattgaaatcaatagccgccactagaggagctactgtagtaattggaacaagcaaattctatggtggttggcacaacatgttaaaaactgtttatagtgatgtagaaaaccctcaccttatgggttgggattatcctaaatgtgatagagccatgcctaacatgcttagaattatggcctcacttgttcttgctcgcaaacatacaacgtgttgtagcttgtcacaccgtttctatagattagctaatgagtgtgctcaagtattgagtgaaatggtcatgtgtggcggttcactatatgttaaaccaggtggaacctcatcaggagatgccacaactgcttatgctaatagtgtttttaacatttgtcaagctgtcacggccaatgttaatgcacttttatctactgatggtaacaaaattgccgataagtatgtccgcaatttacaacacagactttatgagtgtctctatagaaatagagatgttgacacagactttgtgaatgagttttacgcatatttgcgtaaacatttctcaatgatgatactctctgacgatgctgttgtgtgtttcaatagcacttatgcatctcaaggtctagtggctagcataaagaactttaagtcagttctttattatcaaaacaatgtttttatgtctgaagcaaaatgttggactgagactgaccttactaaaggacctcatgaattttgctctcaacatacaatgctagttaaacagggtgatgattatgtgtaccttccttacccagatccatcaagaatcctaggggccggctgttttgtagatgatatcgtaaaaacagatggtacacttatgattgaacggttcgtgtctttagctatagatgcttacccacttactaaacatcctaatcaggagtatgctgatgtctttcatttgtacttacaatacataagaaagctacatgatgagttaacaggacacatgttagacatgtattctgttatgcttactaatgataacacttcaaggtattgggaacctgagttttatgaggctatgtacacaccgcatacagtcttacaggctgttggggcttgtgttctttgcaattcacagacttcattaagatgtggtgcttgcatacgtagaccattcttatgttgtaaatgctgttacgaccatgtcatatcaacatcacataaattagtcttgtctgttaatccgtatgtttgcaatgctccaggttgtgatgtcacagatgtgactcaactttacttaggaggtatgagctattattgtaaatcacataaaccacccattagttttccattgtgtgctaatggacaagtttttggtttatataaaaatacatgtgttggtagcgataatgttactgactttaatgcaattgcaacatgtgactggacaaatgctggtgattacattttagctaacacctgtactgaaagactcaagctttttgcagcagaaacgctcaaagctactgaggagacatttaaactgtcttatggtattgctactgtacgtgaagtgctgtctgacagagaattacatctttcatgggaagttggtaaacctagaccaccacttaaccgaaattatgtctttactggttatcgtgtaactaaaaacagtaaagtacaaataggagagtacacctttgaaaaaggtgactatggtgatgctgttgtttaccgaggtacaacaacttacaaattaaatgttggtgattattttgtgctgacatcacatacagtaatgccattaagtgcacctacactagtgccacaagagcactatgttagaattactggcttatacccaacactcaatatctcagatgagttttctagcaatgttgcaaattatcaaaaggttggtatgcaaaagtattctacactccagggaccacctggtactggtaagagtcattttgctattggcctagctctctactacccttctgctcgcatagtgtatacagcttgctctcatgccgctgttgatgcactatgtgagaaggcattaaaatatttgcctatagataaatgtagtagaattatacctgcacgtgctcgtgtagagtgttttgataaattcaaagtgaattcaacattagaacagtatgtcttttgtactgtaaatgcattgcctgagacgacagcagatatagttgtctttgatgaaatttcaatggccacaaattatgatttgagtgttgtcaatgccagattacgtgctaagcactatgtgtacattggcgaccctgctcaattacctgcaccacgcacattgctaactaagggcacactagaaccagaatatttcaattcagtgtgtagacttatgaaaactataggtccagacatgttcctcggaacttgtcggcgttgtcctgctgaaattgttgacactgtgagtgctttggtttatgataataagcttaaagcacataaagacaaatcagctcaatgctttaaaatgttttataagggtgttatcacgcatgatgtttcatctgcaattaacaggccacaaataggcgtggtaagagaattccttacacgtaaccctgcttggagaaaagctgtctttatttcaccttataattcacagaatgctgtagcctcaaagattttgggactaccaactcaaactgttgattcatcacagggctcagaatatgactatgtcatattcactcaaaccactgaaacagctcactcttgtaatgtaaacagatttaatgttgctattaccagagcaaaagtaggcatactttgcataatgtctgatagagacctttatgacaagttgcaatttacaagtcttgaaattccacgtaggaatgtggcaactttacaagctgaaaatgtaacaggactctttaaagattgtagtaaggtaatcactgggttacatcctacacaggcacctacacacctcagtgttgacactaaattcaaaactgaaggtttatgtgttgacatacctggcatacctaaggacatgacctatagaagactcatctctatgatgggttttaaaatgaattatcaagttaatggttaccctaacatgtttatcacccgcgaagaagctataagacatgtacgtgcatggattggcttcgatgtcgaggggtgtcatgctactagagaagctgttggtaccaatttacctttacagctaggtttttctacaggtgttaacctagttgctgtacctacaggttatgttgatacacctaataatacagatttttccagagttagtgctaaaccaccgcctggagatcaatttaaacacctcataccacttatgtacaaaggacttctttggaatgtagtgcgtataaagattgtacaaatgttaagtgacacacttaaaaatctctctgacagagtcgtatttgtcttatgggcacatggctttgagttgacatctatgaagtattttgtgaaaataggacctgagcgcacctgttgtctatgtgatagacgtgccacatgcttttccactgcttcagacacttatgcctgttggcatcattctattggatttgattacgtctataatccgtttatgattgatgttcaacaatggggttttacaggtaacctacaaagcaaccatgatctgtattgtcaagtccatggtaatgcacatgtagctagttgtgatgcaatcatgactaggtgtctagctgtccacgagtgctttgttaagcgtgttgactggactattgaatatcctataattggtgatgaactgaagattaatgcggcttgtagaaaggttcaacacatggttgttaaagctgcattattagcagacaaattcccagttcttcacgacattggtaaccctaaagctattaagtgtgtacctcaagctgatgtagaatggaagttctatgatgcacagccttgtagtgacaaagcttataaaatagaagaattattctattcttatgccacacattctgacaaattcacagatggtgtatgcctattttggaattgcaatgtcgatagatatcctgctaattccattgtttgtagatttgacactagagtgctatctaaccttaacttgcctggttgtgatggtggcagtttgtatgtaaataaacatgcattccacacaccagcttttgataaaagtgcttttgttaatttaaaacaattaccatttttctattactctgacagtccatgtgagtctcatggaaaacaagtagtgtcagatatagattatgtaccactaaagtctgctacgtgtataacacgttgcaatttaggtggtgctgtctgtagacatcatgctaatgagtacagattgtatctcgatgcttataacatgatgatctcagctggctttagcttgtgggtttacaaacaatttgatacttataacctctggaacacttttacaagacttcagagtttagaaaatgtggcttttaatgttgtaaataagggacactttgatggacaacagggtgaagtaccagtttctatcattaataacactgtttacacaaaagttgatggtgttgatgtagaattgtttgaaaataaaacaacattacctgttaatgtagcatttgagctttgggctaagcgcaacattaaaccagtaccagaggtgaaaatactcaataatttgggtgtggacattgctgctaatactgtgatctgggactacaaaagagatgctccagcacatatatctactattggtgtttgttctatgactgacatagccaagaaaccaactgaaacgatttgtgcaccactcactgtcttttttgatggtagagttgatggtcaagtagacttatttagaaatgcccgtaatggtgttcttattacagaaggtagtgttaaaggtttacaaccatctgtaggtcccaaacaagctagtcttaatggagtcacattaattggagaagccgtaaaaacacagttcaattattataagaaagttgatggtgttgtccaacaattacctgaaacttactttactcagagtagaaatttacaagaatttaaacccaggagtcaaatggaaattgatttcttagaattagctatggatgaattcattgaacggtataaattagaaggctatgccttcgaacatatcgtttatggagattttagtcatagtcagttaggtggtttacatctactgattggactagctaaacgttttaaggaatcaccttttgaattagaagattttattcctatggacagtacagttaaaaactatttcataacagatgcgcaaacaggttcatctaagtgtgtgtgttctgttattgatttattacttgatgattttgttgaaataataaaatcccaagatttatctgtagtttctaaggttgtcaaagtgactattgactatacagaaatttcatttatgctttggtgtaaagatggccatgtagaaacattttacccaaaattacaatctagtcaagcgtggcaaccgggtgttgctatgcctaatctttacaaaatgcaaagaatgctattagaaaagtgtgaccttcaaaattatggtgatagtgcaacattacctaaaggcataatgatgaatgtcgcaaaatatactcaactgtgtcaatatttaaacacattaacattagctgtaccctataatatgagagttatacattttggtgctggttctgataaaggagttgcaccaggtacagctgttttaagacagtggttgcctacgggtacgctgcttgtcgattcagatcttaatgactttgtctctgatgcagattcaactttgattggtgattgtgcaactgtacatacagctaataaatgggatctcattattagtgatatgtacgaccctaagactaaaaatgttacaaaagaaaatgactctaaagagggttttttcacttacatttgtgggtttatacaacaaaagctagctcttggaggttccgtggctataaagataacagaacattcttggaatgctgatctttataagctcatgggacacttcgcatggtggacagcctttgttactaatgtgaatgcgtcatcatctgaagcatttttaattggatgtaattatcttggcaaaccacgcgaacaaatagatggttatgtcatgcatgcaaattacatattttggaggaatacaaatccaattcagttgtcttcctattctttatttgacatgagtaaatttccccttaaattaaggggtactgctgttatgtctttaaaagaaggtcaaatcaatgatatgattttatctcttcttagtaaaggtagacttataattagagaaaacaacagagttgttatttctagtgatgttcttgttaacaactaatgataggcgatcgc

SEQ ID NO: 2 - protein, 2695 aa, Severe acute respiratory syndrome coronavirus 2 (SARS-CoV-2)
RVCGVSAARLTPCGTGTSTDVVYRAFDIYNDKVAGFAKFLKTNCCRFQEKDEDDNLIDSYFVVKRHTFSNYQHEETIYNLLKDCPAVAKHDFFKFRIDGDMVPHISRQRLTKYTMADLVYALRHFDEGNCDTLKEILVTYNCCDDDYFNKKDWYDFVENPDILRVYANLGERVRQALLKTVQFCDAMRNAGIVGVLTLDNQDLNGNWYDFGDFIQTTPGSGVPVVDSYYSLLMPILTLTRALTAESHVDTDLTKPYIKWDLLKYDFTEERLKLFDRYFKYWDQTYHPNCVNCLDDRCILHCANFNVLFSTVFPPTSFGPLVRKIFVDGVPFVVSTGYHFRELGVVHNQDVNLHSSRLSFKELLVYAADPAMHAASGNLLLDKRTTCFSVAALTNNVAFQTVKPGNFNKDFYDFAVSKGFFKEGSSVELKHFFFAQDGNAAISDYDYYRYNLPTMCDIRQLLFVVEVVDKYFDCYDGGCINANQVIVNNLDKSAGFPFNKWGKARLYYDSMSYEDQDALFAYTKRNVIPTITQMNLKYAISAKNRARTVAGVSICSTMTNRQFHQKLLKSIAATRGATVVIGTSKFYGGWHNMLKTVYSDVENPHLMGWDYPKCDRAMPNMLRIMASLVLARKHTTCCSLSHRFYRLANECAQVLSEMVMCGGSLYVKPGGTSSGDATTAYANSVFNICQAVTANVNALLSTDGNKIADKYVRNLQHRLYECLYRNRDVDTDFVNEFYAYLRKHFSMMILSDDAVVCFNSTYASQGLVASIKNFKSVLYYQNNVFMSEAKCWTETDLTKGPHEFCSQHTMLVKQGDDYVYLPYPDPSRILGAGCFVDDIVKTDGTLMIERFVSLAIDAYPLTKHPNQEYADVFHLYLQYIRKLHDELTGHMLDMYSVMLTNDNTSRYWEPEFYEAMYTPHTVLQAVGACVLCNSQTSLRCGACIRRPFLCCKCCYDHVISTSHKLVLSVNPYVCNAPGCDVTDVTQLYLGGMSYYCKSHKPPISFPLCANGQVFGLYKNTCVGSDNVTDFNAIATCDWTNAGDYILANTCTERLKLFAAETLKATEETFKLSYGIATVREVLSDRELHLSWEVGKPRPPLNRNYVFTGYRVTKNSKVQIGEYTFEKGDYGDAVVYRGTTTYKLNVGDYFVLTSHTVMPLSAPTLVPQEHYVRITGLYPTLNISDEFSSNVANYQKVGMQKYSTLQGPPGTGKSHFAIGLALYYPSARIVYTACSHAAVDALCEKALKYLPIDKCSRIIPARARVECFDKFKVNSTLEQYVFCTVNALPETTADIVVFDEISMATNYDLSVVNARLRAKHYVYIGDPAQLPAPRTLLTKGTLEPEYFNSVCRLMKTIGPDMFLGTCRRCPAEIVDTVSALVYDNKLKAHKDKSAQCFKMFYKGVITHDVSSAINRPQIGVVREFLTRNPAWRKAVFISPYNSQNAVASKILGLPTQTVDSSQGSEYDYVIFTQTTETAHSCNVNRFNVAITRAKVGILCIMSDRDLYDKLQFTSLEIPRRNVATLQAENVTGLFKDCSKVITGLHPTQAPTHLSVDTKFKTEGLCVDIPGIPKDMTYRRLISMMGFKMNYQVNGYPNMFITREEAIRHVRAWIGFDVEGCHATREAVGTNLPLQLGFSTGVNLVAVPTGYVDTPNNTDFSRVSAKPPPGDQFKHLIPLMYKGLLWNVVRIKIVQMLSDTLKNLSDRVVFVLWAHGFELTSMKYFVKIGPERTCCLCDRRATCFSTASDTYACWHHSIGFDYVYNPFMIDVQQWGFTGNLQSNHDLYCQVHGNAHVASCDAIMTRCLAVHECFVKRVDWTIEYPIIGDELKINAACRKVQHMVVKAALLADKFPVLHDIGNPKAIKCVPQADVEWKFYDAQPCSDKAYKIEELFYSYATHSDKFTDGVCLFWNCNVDRYPANSIVCRFDTRVLSNLNLPGCDGGSLYVNKHAFHTPAFDKSAFVNLKQLPFFYYSDSPCESHGKQVVSDIDYVPLKSATCITRCNLGGAVCRHHANEYRLYLDAYNMMISAGFSLWVYKQFDTYNLWNTFTRLQSLENVAFNVVNKGHFDGQQGEVPVSIINNTVYTKVDGVDVELFENKTTLPVNVAFELWAKRNIKPVPEVKILNNLGVDIAANTVIWDYKRDAPAHISTIGVCSMTDIAKKPTETICAPLTVFFDGRVDGQVDLFRNARNGVLITEGSVKGLQPSVGPKQASLNGVTLIGEAVKTQFNYYKKVDGVVQQLPETYFTQSRNLQEFKPRSQMEIDFLELAMDEFIERYKLEGYAFEHIVYGDFSHSQLGGLHLLIGLAKRFKESPFELEDFIPMDSTVKNYFITDAQTGSSKCVCSVIDLLLDDFVEIIKSQDLSVVSKVVKVTIDYTEISFMLWCKDGHVETFYPKLQSSQAWQPGVAMPNLYKMQRMLLEKCDLQNYGDSATLPKGIMMNVAKYTQLCQYLNTLTLAVPYNMRVIHFGAGSDKGVAPGTAVLRQWLPTGTLLVDSDLNDFVSDADSTLIGDCATVHTANKWDLIISDMYDPKTKNVTKENDSKEGFFTYICGFIQQKLALGGSVAIKITEHSWNADLYKLMGHFAWWTAFVTNVNASSSEAFLIGCNYLGKPREQIDGYVMHANYIFWRNTNPIQLSSYSLFDMSKFPLKLRGTAVMSLKEGQINDMILSLLSKGRLIIRENNRVVISSDVLVNN

SEQ ID NO: 3 - DNA, 8198 bp, Artificial
  Synthetic DNA
  CDS (97)..(8181)
cctgcaggaaaaattgaaaataaatacaaaggttcttgagggttgtgttaaattgaaagcgagaaataatcataaatatgaccgaaaggtaagatgcgggtttgcggtgtaagtgcagcccgtcttacaccgtgcggcacaggcactagtactgatgtcgtatacagggcttttgacatctacaatgataaagtagctggttttgctaaattcctaaaaactaattgttgtcgcttccaagaaaaggacgaagatgacaatttaattgattcttactttgtagttaagagacacactttctctaactaccaacatgaagaaacaatttataatttacttaaggattgtccagctgttgctaaacatgacttctttaagtttagaatagacggtgacatggtaccacatatatcacgtcaacgtcttactaaatacacaatggcagacctcgtctatgctttaaggcattttgatgaaggtaattgtgacacattaaaagaaatacttgtcacatacaattgttgtgatgatgattatttcaataaaaaggactggtatgattttgtagaaaacccagatatattacgcgtatacgccaacttaggtgaacgtgtacgccaagctttgttaaaaacagtacaattctgtgatgccatgcgaaatgctggtattgttggtgtactgacattagataatcaagatctcaatggtaactggtatgatttcggtgatttcatacaaaccacgccaggtagtggagttcctgttgtagattcttattattcattgttaatgcctatattaaccttgaccagggctttaactgcagagtcacatgttgacactgacttaacaaagccttacattaagtgggatttgttaaaatatgacttcacggaagagaggttaaaactctttgaccgttattttaaatattgggatcagacataccacccaaattgtgttaactgtttggatgacagatgcattctgcattgtgcaaactttaatgttttattctctacagtgttcccacctacaagttttggaccactagtgagaaaaatatttgttgatggtgttccatttgtagtttcaactggataccacttcagagagctaggtgttgtacataatcaggatgtaaacttacatagctctagacttagttttaaggaattacttgtgtatgctgctgaccctgctatgcacgctgcttctggtaatctattactagataaacgcactacgtgcttttcagtagctgcacttactaacaatgttgcttttcaaactgtcaaacccggtaattttaacaaagacttctatgactttgctgtgtctaagggtttctttaaggaaggaagttctgttgaattaaaacacttcttctttgctcaggatggtaatgctgctatcagcgattatgactactatcgttataatctaccaacaatgtgtgatatcagacaactactatttgtagttgaagttgttgataagtactttgattgttacgatggtggctgtattaatgctaaccaagtcatcgtcaacaacctagacaaatcagctggttttccatttaataaatggggtaaggctagactttattatgattcaatgagttatgaggatcaagatgcacttttcgcatatacaaaacgtaatgtcatccctactataactcaaatgaatcttaagtatgccattagtgcaaagaatagagctcgcaccgtagctggtgtctctatctgtagtactatgaccaatagacagtttcatcaaaaattattgaaatcaatagccgccactagaggagctactgtagtaattggaacaagcaaattctatggtggttggcacaacatgttaaaaactgtttatagtgatgtagaaaaccctcaccttatgggttgggattatcctaaatgtgatagagccatgcctaacatgcttagaattatggcctcacttgttcttgctcgcaaacatacaacgtgttgtagcttgtcacaccgtttctatagattagctaatgagtgtgctcaagtattgagtgaaatggtcatgtgtggcggttcactatatgttaaaccaggtggaacctcatcaggagatgccacaactgcttatgctaatagtgtttttaacatttgtcaagctgtcacggccaatgttaatgcacttttatctactgatggtaacaaaattgccgataagtatgtccgcaatttacaacacagactttatgagtgtctctatagaaatagagatgttgacacagactttgtgaatgagttttacgcatatttgcgtaaacatttctcaatgatgatactctctgacgatgctgttgtgtgtttcaatagcacttatgcatctcaaggtctagtggctagcataaagaactttaagtcagttctttattatcaaaacaatgtcttcatgtctgaagcaaaatgttggactgagactgaccttactaaaggacctcatgaattttgctctcaacatacaatgctagttaaacagggtaatgattatgtgtaccttccttacccagatccatcaagaatcctaggggccggctgttttgtagatgatatcgtaaaaacagatggtacacttatgattgaacggttcgtgtctttagctatagatgcttacccacttactaaacatcctaatcaggagtatgctgatgtctttcatttgtacttacaatacataagaaagctacatgatgagttaacaggacacatgttagacatgtattctgttatgcttactaatgataacacttcaaggtattgggaacctgagttttatgaggctatgtacacaccgcatacagtcttacaggctgttggggcttgtgttctttgcaattcacagacttcattaagatgtggtgcttgcatacgtagaccattcttatgttgtaaatgctgttacgaccatgtcatatcaacatcacataaattagtcttgtctgttaatccgtatgtttgcaatgctccaggttgtgatgtcacagatgtgactcaactttacttaggaggtatgagctattattgtaaatcacataaaccacccattagttttccattgtgtgctaatggacaagtttttggtttatataaaaatacatgtgttggtagcgataatgttactgactttaatgcaattgcaacatgtgactggacaaatgctggtgattacattttagctaacacctgtactgaaagactcaagctttttgcagcagaaacgctcaaagctactgaggagacatttaaactgtcttatggtattgctactgtacgtgaagtgctgtctgacagagaattacatctttcatgggaagttggtaaacctagaccaccacttaaccgaaattatgtctttactggttatcgtgtaactaaaaacagtaaagtacaaataggagagtacacctttgaaaaaggtgactatggtgatgctgttgtttaccgaggtacaacaacttacaaattaaatgttggtgattattttgtgctgacatcacatacagtaatgccattaagtgcacctacactagtgccacaagagcactatgttagaattactggcttatacccaacactcaatatctcagatgagttttctagcaatgttgcaaattatcaaaaggttggtatgcaaaagtattctacactccagggaccacctggtactggtaagagtcattttgctattggcctagctctctactacccttctgctcgcatagtgtatacagcttgctctcatgccgctgttgatgcactatgtgagaaggcattaaaatatttgcctatagataaatgtagtagaattatacctgcacgtgctcgtgtagagtgttttgataaattcaaagtgaattcaacattagaacagtatgtcttttgtactgtaaatgcattgcctgagacgacagcagatatagttgtctttgatgaaatttcaatggccacaaattatgatttgagtgttgtcaatgccagattacgtgctaagcactatgtgtacattggcgaccctgctcaattacctgcaccacgcacattgctaactaagggcacactagaaccagaatatttcaattcagtgtgtagacttatgaaaactataggtccagacatgttcctcggaacttgtcggcgttgtcctgctgaaattgttgacactgtgagtgctttggtttatgataataagcttaaagcacataaagacaaatcagctcaatgctttaaaatgttttataagggtgttatcacgcatgatgtttcatctgcaattaacaggccacaaataggcgtggtaagagaattccttacacgtaaccctgcttggagaaaagctgtctttatttcaccttataattcacagaatgctgtagcctcaaagattttgggactaccaactcaaactgttgattcatcacagggctcagaatatgactatgtcatattcactcaaaccactgaaacagctcactcttgtaatgtaaacagatttaatgttgctattaccagagcaaaagtaggcatactttgcataatgtctgatagagacctttatgacaagttgcaatttacaagtcttgaaattccacgtaggaatgtggcaactttacaagctgaaaatgtaacaggactctttaaagattgtagtaaggtaatcactgggttacatcctacacaggcacctacacacctcagtgttgacactaaattcaaaactgaaggtttatgtgttgacatacctggcatacctaaggacatgacctatagaagactcatctctatgatgggttttaaaatgaattatcaagttaatggttaccctaacatgtttatcacccgcgaagaagctataagacatgtacgtgcatggattggcttcgatgtcgaggggtgtcatgctactagagaagctgttggtaccaatttacctttacagctaggcttctctacaggtgttaacctagttgctgtacctacaggttatgttgatacacctaataatacagatttttccagagttagtgctaaaccaccgcctggagatcaatttaaacacctcataccacttatgtacaaaggacttctttggaatgtagtgcgtataaagattgtacaaatgttaagtgacacacttaaaaatctctctgacagagtcgtatttgtcttatgggcacatggctttgagttgacatctatgaagtattttgtgaaaataggacctgagcgcacctgttgtctatgtgatagacgtgccacatgcttttccactgcttcagacacttatgcctgttggcatcattctattggatttgattacgtctataatccgtttatgattgatgttcaacaatggggttttacaggtaacctacaaagcaaccatgatctgtattgtcaagtccatggtaatgcacatgtagctagttgtgatgcaatcatgactaggtgtctagctgtccacgagtgctttgttaagcgtgttgactggactattgaatatcctataattggtgatgaactgaagattaatgcggcttgtagaaaggttcaacacatggttgttaaagctgcattattagcagacaaattcccagttcttcacgacattggtaaccctaaagctattaagtgtgtacctcaagctgatgtagaatggaagttctatgatgcacagccttgtagtgacaaagcttataaaatagaagaattattctattcttatgccacacattctgacaaattcacagatggtgtatgcctattttggaattgcaatgtcgatagatatcctgctaattccattgtttgtagatttgacactagagtgctatctaaccttaacttgcctggttgtgatggtggcagtttgtatgtaaataaacatgcattccacacaccagcttttgataaaagtgcttttgttaatttaaaacaattaccattcttctattactctgacagtccatgtgagtctcatggaaaacaagtagtgtcagatatagattatgtaccactaaagtctgctacgtgtataacacgttgcaatttaggtggtgctgtctgtagacatcatgctaatgagtacagattgtatctcgatgcttataacatgatgatctcagctggctttagcttgtgggtttacaaacaatttgatacttataacctctggaacacttttacaagacttcagagtttagaaaatgtggcttttaatgttgtaaataagggacactttgatggacaacagggtgaagtaccagtttctatcattaataacactgtttacacaaaagttgatggtgttgatgtagaattgtttgaaaataaaacaacattacctgttaatgtagcatttgagctttgggctaagcgcaacattaaaccagtaccagaggtgaaaatactcaataatttgggtgtggacattgctgctaatactgtgatctgggactacaaaagagatgctccagcacatatatctactattggtgtttgttctatgactgacatagccaagaaaccaactgaaacgatttgtgcaccactcactgtcttttttgatggtagagttgatggtcaagtagacttatttagaaatgcccgtaatggtgttcttattacagaaggtagtgttaaaggtttacaaccatctgtaggtcccaaacaagctagtcttaatggagtcacattaattggagaagccgtaaaaacacagttcaattattataagaaagttgatggtgttgtccaacaattacctgaaacttactttactcagagtagaaatttacaagaatttaaacccaggagtcaaatggaaattgatttcttagaattagctatggatgaattcattgaacggtataaattagaaggctatgccttcgaacatatcgtttatggagattttagtcatagtcagttaggtggtttacatctactgattggactagctaaacgttttaaggaatcaccttttgaattagaagattttattcctatggacagtacagttaaaaactatttcataacagatgcgcaaacaggttcatctaagtgtgtgtgttctgttattgatttattacttgatgattttgttgaaataataaaatcccaagatttatctgtagtttctaaggttgtcaaagtgactattgactatacagaaatttcatttatgctttggtgtaaagatggccatgtagaaacattttacccaaaattacaatctagtcaagcgtggcaaccgggtgttgctatgcctaatctttacaaaatgcaaagaatgctattagaaaagtgtgaccttcaaaattatggtgatagtgcaacattacctaaaggcataatgatgaatgtcgcaaaatatactcaactgtgtcaatatttaaacacattaacattagctgtaccctataatatgagagttatacattttggtgctggttctgataaaggagttgcaccaggtacagctgttttaagacagtggttgcctacgggtacgctgcttgtcgattcagatcttaatgactttgtctctgatgcagattcaactttgattggtgattgtgcaactgtacatacagctaataaatgggatctcattattagtgatatgtacgaccctaagactaaaaatgttacaaaagaaaatgactctaaagagggttttttcacttacatttgtgggtttatacaacaaaagctagctcttggaggttccgtggctataaagataacagaacattcttggaatgctgatctttataagctcatgggacacttcgcatggtggacagcctttgttactaatgtgaatgcgtcatcatctgaagcatttttaattggatgtaattatcttggcaaaccacgcgaacaaatagatggttatgtcatgcatgcaaattacatattttggaggaatacaaatccaattcagttgtcttcctattctttatttgacatgagtaaatttccccttaaattaaggggtactgctgttatgtctttaaaagaaggtcaaatcaatgatatgattttatctcttcttagtaaaggtagacttataattagagaaaacaacagagttgttatttctagtgatgttcttgttaacaactaatgataggcgatcgc

SEQ ID NO: 4 - protein, 2695 aa, Artificial
  Synthetic Construct
RVCGVSAARLTPCGTGTSTDVVYRAFDIYNDKVAGFAKFLKTNCCRFQEKDEDDNLIDSYFVVKRHTFSNYQHEETIYNLLKDCPAVAKHDFFKFRIDGDMVPHISRQRLTKYTMADLVYALRHFDEGNCDTLKEILVTYNCCDDDYFNKKDWYDFVENPDILRVYANLGERVRQALLKTVQFCDAMRNAGIVGVLTLDNQDLNGNWYDFGDFIQTTPGSGVPVVDSYYSLLMPILTLTRALTAESHVDTDLTKPYIKWDLLKYDFTEERLKLFDRYFKYWDQTYHPNCVNCLDDRCILHCANFNVLFSTVFPPTSFGPLVRKIFVDGVPFVVSTGYHFRELGVVHNQDVNLHSSRLSFKELLVYAADPAMHAASGNLLLDKRTTCFSVAALTNNVAFQTVKPGNFNKDFYDFAVSKGFFKEGSSVELKHFFFAQDGNAAISDYDYYRYNLPTMCDIRQLLFVVEVVDKYFDCYDGGCINANQVIVNNLDKSAGFPFNKWGKARLYYDSMSYEDQDALFAYTKRNVIPTITQMNLKYAISAKNRARTVAGVSICSTMTNRQFHQKLLKSIAATRGATVVIGTSKFYGGWHNMLKTVYSDVENPHLMGWDYPKCDRAMPNMLRIMASLVLARKHTTCCSLSHRFYRLANECAQVLSEMVMCGGSLYVKPGGTSSGDATTAYANSVFNICQAVTANVNALLSTDGNKIADKYVRNLQHRLYECLYRNRDVDTDFVNEFYAYLRKHFSMMILSDDAVVCFNSTYASQGLVASIKNFKSVLYYQNNVFMSEAKCWTETDLTKGPHEFCSQHTMLVKQGNDYVYLPYPDPSRILGAGCFVDDIVKTDGTLMIERFVSLAIDAYPLTKHPNQEYADVFHLYLQYIRKLHDELTGHMLDMYSVMLTNDNTSRYWEPEFYEAMYTPHTVLQAVGACVLCNSQTSLRCGACIRRPFLCCKCCYDHVISTSHKLVLSVNPYVCNAPGCDVTDVTQLYLGGMSYYCKSHKPPISFPLCANGQVFGLYKNTCVGSDNVTDFNAIATCDWTNAGDYILANTCTERLKLFAAETLKATEETFKLSYGIATVREVLSDRELHLSWEVGKPRPPLNRNYVFTGYRVTKNSKVQIGEYTFEKGDYGDAVVYRGTTTYKLNVGDYFVLTSHTVMPLSAPTLVPQEHYVRITGLYPTLNISDEFSSNVANYQKVGMQKYSTLQGPPGTGKSHFAIGLALYYPSARIVYTACSHAAVDALCEKALKYLPIDKCSRIIPARARVECFDKFKVNSTLEQYVFCTVNALPETTADIVVFDEISMATNYDLSVVNARLRAKHYVYIGDPAQLPAPRTLLTKGTLEPEYFNSVCRLMKTIGPDMFLGTCRRCPAEIVDTVSALVYDNKLKAHKDKSAQCFKMFYKGVITHDVSSAINRPQIGVVREFLTRNPAWRKAVFISPYNSQNAVASKILGLPTQTVDSSQGSEYDYVIFTQTTETAHSCNVNRFNVAITRAKVGILCIMSDRDLYDKLQFTSLEIPRRNVATLQAENVTGLFKDCSKVITGLHPTQAPTHLSVDTKFKTEGLCVDIPGIPKDMTYRRLISMMGFKMNYQVNGYPNMFITREEAIRHVRAWIGFDVEGCHATREAVGTNLPLQLGFSTGVNLVAVPTGYVDTPNNTDFSRVSAKPPPGDQFKHLIPLMYKGLLWNVVRIKIVQMLSDTLKNLSDRVVFVLWAHGFELTSMKYFVKIGPERTCCLCDRRATCFSTASDTYACWHHSIGFDYVYNPFMIDVQQWGFTGNLQSNHDLYCQVHGNAHVASCDAIMTRCLAVHECFVKRVDWTIEYPIIGDELKINAACRKVQHMVVKAALLADKFPVLHDIGNPKAIKCVPQADVEWKFYDAQPCSDKAYKIEELFYSYATHSDKFTDGVCLFWNCNVDRYPANSIVCRFDTRVLSNLNLPGCDGGSLYVNKHAFHTPAFDKSAFVNLKQLPFFYYSDSPCESHGKQVVSDIDYVPLKSATCITRCNLGGAVCRHHANEYRLYLDAYNMMISAGFSLWVYKQFDTYNLWNTFTRLQSLENVAFNVVNKGHFDGQQGEVPVSIINNTVYTKVDGVDVELFENKTTLPVNVAFELWAKRNIKPVPEVKILNNLGVDIAANTVIWDYKRDAPAHISTIGVCSMTDIAKKPTETICAPLTVFFDGRVDGQVDLFRNARNGVLITEGSVKGLQPSVGPKQASLNGVTLIGEAVKTQFNYYKKVDGVVQQLPETYFTQSRNLQEFKPRSQMEIDFLELAMDEFIERYKLEGYAFEHIVYGDFSHSQLGGLHLLIGLAKRFKESPFELEDFIPMDSTVKNYFITDAQTGSSKCVCSVIDLLLDDFVEIIKSQDLSVVSKVVKVTIDYTEISFMLWCKDGHVETFYPKLQSSQAWQPGVAMPNLYKMQRMLLEKCDLQNYGDSATLPKGIMMNVAKYTQLCQYLNTLTLAVPYNMRVIHFGAGSDKGVAPGTAVLRQWLPTGTLLVDSDLNDFVSDADSTLIGDCATVHTANKWDLIISDMYDPKTKNVTKENDSKEGFFTYICGFIQQKLALGGSVAIKITEHSWNADLYKLMGHFAWWTAFVTNVNASSSEAFLIGCNYLGKPREQIDGYVMHANYIFWRNTNPIQLSSYSLFDMSKFPLKLRGTAVMSLKEGQINDMILSLLSKGRLIIRENNRVVISSDVLVNN

SEQ ID NO: 5 - DNA, 3926 bp, Severe acute respiratory syndrome coronavirus 2 (SARS-CoV-2)
  CDS (91)..(3909)
cctgcaggaaaaattgaaaataaatacaaaggttcttgagggttgtgttaaattgaaagcgagaaataatcataaataactaaacgaacaatgtttgtttttcttgttttattgccactagtctctagtcagtgtgttaatcttacaaccagaactcaattaccccctgcatacactaattctttcacacgtggtgtttattaccctgacaaagttttcagatcctcagttttacattcaactcaggacttgttcttacctttcttttccaatgttacttggttccatgctatacatgtctctgggaccaatggtactaagaggtttgataaccctgtcctaccatttaatgatggtgtttattttgcttccactgagaagtctaacataataagaggctggatttttggtactactttagattcgaagacccagtccctacttattgttaataacgctactaatgttgttattaaagtctgtgaatttcaattttgtaatgatccatttttgggtgtttattaccacaaaaacaacaaaagttggatggaaagtgagttcagagtttattctagtgcgaataattgcacttttgaatatgtctctcagccttttcttatggaccttgaaggaaaacagggtaatttcaaaaatcttagggaatttgtgtttaagaatattgatggttattttaaaatatattctaagcacacgcctattaatttagtgcgtgatctccctcagggtttttcggctttagaaccattggtagatttgccaataggtattaacatcactaggtttcaaactttacttgctttacatagaagttatttgactcctggtgattcttcttcaggttggacagctggtgctgcagcttattatgtgggttatcttcaacctaggacttttctattaaaatataatgaaaatggaaccattacagatgctgtagactgtgcacttgaccctctctcagaaacaaagtgtacgttgaaatccttcactgtagaaaaaggaatctatcaaacttctaactttagagtccaaccaacagaatctattgttagatttcctaatattacaaacttgtgcccttttggtgaagtttttaacgccaccagatttgcatctgtttatgcttggaacaggaagagaatcagcaactgtgttgctgattattctgtcctatataattccgcatcattttccacttttaagtgttatggagtgtctcctactaaattaaatgatctctgctttactaatgtctatgcagattcatttgtaattagaggtgatgaagtcagacaaatcgctccagggcaaactggaaagattgctgattataattataaattaccagatgattttacaggctgcgttatagcttggaattctaacaatcttgattctaaggttggtggtaattataattacctgtatagattgtttaggaagtctaatctcaaaccttttgagagagatatttcaactgaaatctatcaggccggtagcacaccttgtaatggtgttgaaggttttaattgttactttcctttacaatcatatggtttccaacccactaatggtgttggttaccaaccatacagagtagtagtactttcttttgaacttctacatgcaccagcaactgtttgtggacctaaaaagtctactaatttggttaaaaacaaatgtgtcaatttcaacttcaatggtttaacaggcacaggtgttcttactgagtctaacaaaaagtttctgcctttccaacaatttggcagagacattgctgacactactgatgctgtccgtgatccacagacacttgagattcttgacattacaccatgttcttttggtggtgtcagtgttataacaccaggaacaaatacttctaaccaggttgctgttctttatcaggatgttaactgcacagaagtccctgttgctattcatgcagatcaacttactcctacttggcgtgtttattctacaggttctaatgtttttcaaacacgtgcaggctgtttaataggggctgaacatgtcaacaactcatatgagtgtgacatacccattggtgcaggtatatgcgctagttatcagactcagactaattctcctcggcgggcacgtagtgtagctagtcaatccatcattgcctacactatgtcacttggtgcagaaaattcagttgcttactctaataactctattgccatacccacaaattttactattagtgttaccacagaaattctaccagtgtctatgaccaagacatcagtagattgtacaatgtacatttgtggtgattcaactgaatgcagcaatcttttgttgcaatatggcagtttttgtacacaattaaaccgtgctttaactggaatagctgttgaacaagacaaaaacacccaagaagtttttgcacaagtcaaacaaatttacaaaacaccaccaattaaagattttggtggttttaatttttcacaaatattaccagatccatcaaaaccaagcaagaggtcatttattgaagatctacttttcaacaaagtgacacttgcagatgctggcttcatcaaacaatatggtgattgccttggtgatattgctgctagagacctcatttgtgcacaaaagtttaacggccttactgttttgccacctttgctcacagatgaaatgattgctcaatacacttctgcactgttagcgggtacaatcacttctggttggacctttggtgcaggtgctgcattacaaataccatttgctatgcaaatggcttataggtttaatggtattggagttacacagaatgttctctatgagaaccaaaaattgattgccaaccaatttaatagtgctattggcaaaattcaagactcactttcttccacagcaagtgcacttggaaaacttcaagatgtggtcaaccaaaatgcacaagctttaaacacgcttgttaaacaacttagctccaattttggtgcaatttcaagtgttttaaatgatatcctttcacgtcttgacaaagttgaggctgaagtgcaaattgataggttgatcacaggcagacttcaaagtttgcagacatatgtgactcaacaattaattagagctgcagaaatcagagcttctgctaatcttgctgctactaaaatgtcagagtgtgtacttggacaatcaaaaagagttgatttttgtggaaagggctatcatcttatgtccttccctcagtcagcacctcatggtgtagtcttcttgcatgtgacttatgtccctgcacaagaaaagaacttcacaactgctcctgccatttgtcatgatggaaaagcacactttcctcgtgaaggtgtctttgtttcaaatggcacacactggtttgtaacacaaaggaatttttatgaaccacaaatcattactacagacaacacatttgtgtctggtaactgtgatgttgtaataggaattgtcaacaacacagtttatgatcctttgcaacctgaattagactcattcaaggaggagttagataaatattttaagaatcatacatcaccagatgttgatttaggtgacatctctggcattaatgcttcagttgtaaacattcaaaaagaaattgaccgcctcaatgaggttgccaagaatttaaatgaatctctcatcgatctccaagaacttggaaagtatgagcagtatataaaatggccatggtacatttggctaggttttatagctggcttgattgccatagtaatggtgacaattatgctttgctgtatgaccagttgctgtagttgtctcaagggctgttgttcttgtggatcctgctgcaaatttgatgaagacgactctgagccagtgctcaaaggagtcaaattacattacacataatgataggcgatcgc

SEQ ID NO: 6 - protein, 1273 aa, Severe acute respiratory syndrome coronavirus 2 (SARS-CoV-2)
MFVFLVLLPLVSSQCVNLTTRTQLPPAYTNSFTRGVYYPDKVFRSSVLHSTQDLFLPFFSNVTWFHAIHVSGTNGTKRFDNPVLPFNDGVYFASTEKSNIIRGWIFGTTLDSKTQSLLIVNNATNVVIKVCEFQFCNDPFLGVYYHKNNKSWMESEFRVYSSANNCTFEYVSQPFLMDLEGKQGNFKNLREFVFKNIDGYFKIYSKHTPINLVRDLPQGFSALEPLVDLPIGINITRFQTLLALHRSYLTPGDSSSGWTAGAAAYYVGYLQPRTFLLKYNENGTITDAVDCALDPLSETKCTLKSFTVEKGIYQTSNFRVQPTESIVRFPNITNLCPFGEVFNATRFASVYAWNRKRISNCVADYSVLYNSASFSTFKCYGVSPTKLNDLCFTNVYADSFVIRGDEVRQIAPGQTGKIADYNYKLPDDFTGCVIAWNSNNLDSKVGGNYNYLYRLFRKSNLKPFERDISTEIYQAGSTPCNGVEGFNCYFPLQSYGFQPTNGVGYQPYRVVVLSFELLHAPATVCGPKKSTNLVKNKCVNFNFNGLTGTGVLTESNKKFLPFQQFGRDIADTTDAVRDPQTLEILDITPCSFGGVSVITPGTNTSNQVAVLYQDVNCTEVPVAIHADQLTPTWRVYSTGSNVFQTRAGCLIGAEHVNNSYECDIPIGAGICASYQTQTNSPRRARSVASQSIIAYTMSLGAENSVAYSNNSIAIPTNFTISVTTEILPVSMTKTSVDCTMYICGDSTECSNLLLQYGSFCTQLNRALTGIAVEQDKNTQEVFAQVKQIYKTPPIKDFGGFNFSQILPDPSKPSKRSFIEDLLFNKVTLADAGFIKQYGDCLGDIAARDLICAQKFNGLTVLPPLLTDEMIAQYTSALLAGTITSGWTFGAGAALQIPFAMQMAYRFNGIGVTQNVLYENQKLIANQFNSAIGKIQDSLSSTASALGKLQDVVNQNAQALNTLVKQLSSNFGAISSVLNDILSRLDKVEAEVQIDRLITGRLQSLQTYVTQQLIRAAEIRASANLAATKMSECVLGQSKRVDFCGKGYHLMSFPQSAPHGVVFLHVTYVPAQEKNFTTAPAICHDGKAHFPREGVFVSNGTHWFVTQRNFYEPQIITTDNTFVSGNCDVVIGIVNNTVYDPLQPELDSFKEELDKYFKNHTSPDVDLGDISGINASVVNIQKEIDRLNEVAKNLNESLIDLQELGKYEQYIKWPWYIWLGFIAGLIAIVMVTIMLCCMTSCCSCLKGCCSCGSCCKFDEDDSEPVLKGVKLHYT

SEQ ID NO: 7 - DNA, 3926 bp, Artificial
  Synthetic DNA
  CDS (91)..(3909)
cctgcaggaaaaattgaaaataaatacaaaggttcttgagggttgtgttaaattgaaagcgagaaataatcataaataactaaacgaacaatgtttgtcttccttgttttattgccactagtctctagtcagtgtgttaatcttacaaccagaactcaattaccccctgcatacactaattctttcacacgtggtgtttattaccctgacaaagttttcagatcctcagttttacattcaactcaggacttgttcttacctttcttttccaatgttacttggttccatgctatacatgtctctgggaccaatggtactaagaggtttgataaccctgtcctaccatttaatgatggtgtttattttgcttccactgagaagtctaacataataagaggctggatttttggtactactttagattcgaagacccagtccctacttattgttaataacgctactaatgttgttattaaagtctgtgaatttcaattttgtaatgatccatttttgggtgtttattaccacaaaaacaacaaaagttggatggaaagtgagttcagagtttattctagtgcgaataattgcacttttgaatatgtctctcagccttttcttatggaccttgaaggaaaacagggtaatttcaaaaatcttagggaatttgtgtttaagaatattgatggttattttaaaatatattctaagcacacgcctattaatttagtgcgtgatctccctcagggtttttcggctttagaaccattggtagatttgccaataggtattaacatcactaggtttcaaactttacttgctttacatagaagttatttgactcctggtgattcttcttcaggttggacagctggtgctgcagcttattatgtgggttatcttcaacctaggacttttctattaaaatataatgaaaatggaaccattacagatgctgtagactgtgcacttgaccctctctcagaaacaaagtgtacgttgaaatccttcactgtagaaaaaggaatctatcaaacttctaactttagagtccaaccaacagaatctattgttagatttcctaatattacaaacttgtgcccttttggtgaagtttttaacgccaccagatttgcatctgtttatgcttggaacaggaagagaatcagcaactgtgttgctgattattctgtcctatataattccgcatcattttccacttttaagtgttatggagtgtctcctactaaattaaatgatctctgctttactaatgtctatgcagattcatttgtaattagaggtgatgaagtcagacaaatcgctccagggcaaactggaaagattgctgattataattataaattaccagatgattttacaggctgcgttatagcttggaattctaacaatcttgattctaaggttggtggtaattataattacctgtatagattgtttaggaagtctaatctcaaaccttttgagagagatatttcaactgaaatctatcaggccggtagcacaccttgtaatggtgttgaaggttttaattgttactttcctttacaatcatatggtttccaacccactaatggtgttggttaccaaccatacagagtagtagtactttcttttgaacttctacatgcaccagcaactgtttgtggacctaaaaagtctactaatttggttaaaaacaaatgtgtcaatttcaacttcaatggtttaacaggcacaggtgttcttactgagtctaacaaaaagtttctgcctttccaacaatttggcagagacattgctgacactactgatgctgtccgtgatccacagacacttgagattcttgacattacaccatgttcttttggtggtgtcagtgttataacaccaggaacaaatacttctaaccaggttgctgttctttatcaggatgttaactgcacagaagtccctgttgctattcatgcagatcaacttactcctacttggcgtgtttattctacaggttctaatgtttttcaaacacgtgcaggctgtttaataggggctgaacatgtcaacaactcatatgagtgtgacatacccattggtgcaggtatatgcgctagttatcagactcagactaattctcctcggcgggcacgtagtgtagctagtcaatccatcattgcctacactatgtcacttggtgcagaaaattcagttgcttactctaataactctattgccatacccacaaattttactattagtgttaccacagaaattctaccagtgtctatgaccaagacatcagtagattgtacaatgtacatttgtggtgattcaactgaatgcagcaatcttttgttgcaatatggcagcttctgtacacaattaaaccgtgctttaactggaatagctgttgaacaagacaaaaacacccaagaagtttttgcacaagtcaaacaaatttacaaaacaccaccaattaaagattttggtggttttaatttttcacaaatattaccagatccatcaaaaccaagcaagaggtcatttattgaagatctacttttcaacaaagtgacacttgcagatgctggcttcatcaaacaatatggtgattgccttggtgatattgctgctagagacctcatttgtgcacaaaagtttaacggccttactgttttgccacctttgctcacagatgaaatgattgctcaatacacttctgcactgttagcgggtacaatcacttctggttggacctttggtgcaggtgctgcattacaaataccatttgctatgcaaatggcttataggtttaatggtattggagttacacagaatgttctctatgagaaccaaaaattgattgccaaccaatttaatagtgctattggcaaaattcaagactcactttcttccacagcaagtgcacttggaaaacttcaagatgtggtcaaccaaaatgcacaagctttaaacacgcttgttaaacaacttagctccaattttggtgcaatttcaagtgttttaaatgatatcctttcacgtcttgacaaagttgaggctgaagtgcaaattgataggttgatcacaggcagacttcaaagtttgcagacatatgtgactcaacaattaattagagctgcagaaatcagagcttctgctaatcttgctgctactaaaatgtcagagtgtgtacttggacaatcaaaaagagttgacttctgtggaaagggctatcatcttatgtccttccctcagtcagcacctcatggtgtagtcttcttgcatgtgacttatgtccctgcacaagaaaagaacttcacaactgctcctgccatttgtcatgatggaaaagcacactttcctcgtgaaggtgtctttgtttcaaatggcacacactggtttgtaacacaaaggaatttctacgaaccacaaatcattactacagacaacacatttgtgtctggtaactgtgatgttgtaataggaattgtcaacaacacagtttatgatcctttgcaacctgaattagactcattcaaggaggagttagataaatattttaagaatcatacatcaccagatgttgatttaggtgacatctctggcattaatgcttcagttgtaaacattcaaaaagaaattgaccgcctcaatgaggttgccaagaatttaaatgaatctctcatcgatctccaagaacttggaaagtatgagcagtatataaaatggccatggtacatttggctaggttttatagctggcttgattgccatagtaatggtgacaattatgctttgctgtatgaccagttgctgtagttgtctcaagggctgttgttcttgtggatcctgctgcaaatttgatgaagacgactctgagccagtgctcaaaggagtcaaattacattacacataatgataggcgatcgc

SEQ ID NO: 8 - protein, 1273 aa, Artificial; identical to SEQ ID NO: 6
  Synthetic Construct

SEQ ID NO: 9 - DNA, 29848 bp, Severe acute respiratory syndrome coronavirus 2 (SARS-CoV-2)
aaaggtttataccttcccaggtaacaaaccaaccaactttcgatctcttgtagatctgttctctaaacgaactttaaaatctgtgtggctgtcactcggctgcatgcttagtgcactcacgcagtataattaataactaattactgtcgttgacaggacacgagtaactcgtctatcttctgcaggctgcttacggtttcgtccgtgttgcagccgatcatcagcacatctaggtttcgtccgggtgtgaccgaaaggtaagatggagagccttgtccctggtttcaacgagaaaacacacgtccaactcagtttgcctgttttacaggttcgcgacgtgctcgtacgtggcttttcagaggcacgtcaacatcttaaagatggcacttgtggcttagtagaagttgaaaaaggcgttttgcctcaacttgaacagccctatgtgttcatcaaacgttcggatgctcgaactgcacctcatggtcatgttatggttgagctggtagcagaactcgaaggcattcagtacggtcgtagtggtgagacacttggtgtccttgtccctcatgtgggcgaaataccagtggcttaccgcaaggttcttcttcgtaagaacggtaataaaggagctggtggccatagttacggcgccgatctaaagtcatttgacttaggcgacgagcttggcactgatccttatgaagattttcaagaaaactggaacactaaacatagcagtggtgttacccgtgaactcatgcgtgagcttaacggaggggcatacactcgctatgtcgataacaacttctgtggccctgatggctaccctcttgagtgcattaaagaccttctagcacgtgctggtaaagcttcatgcactttgtccgaacaactggactttattgacactaagaggggtgtatactgctgccgtgaacatgagcatgaaattgcttggtacacggaacgttctgaaaagagctatgaattgcagacaccttttgaaattaaattggcaaagaaatttgacaccttcaatggggaatgtccaaattttgtatttcccttaaattccataatcaagactattcaaccaagggttgaaaagaaaaagcttgatggctttatgggtagaattcgatctgtctatccagttgcgtcaccaaatgaatgcaaccaaatgtgcctttcaactctcatgaagtgtgatcattgtggtgaaacttcatggcagacgggcgattttgttaaagccacttgcgaattttgtggcactgagaatttgactaaagaaggtgccactacttgtggttacttaccccaaaatgctgttgttaaaatttattgtccagcatgtcacaattcagaagtaggacctgagcatagtcttgccgaataccataatgaatctggcttgaaaaccattcttcgtaagggtggtcgcactattgcctttggaggctgtgtgttctcttatgttggttgccataacaagtgtgcctattgggttccacgtgctagcgctaacataggttgtaaccatacaggtgttgttggagaaggttccgaaggtcttaatgacaaccttcttgaaatactccaaaaagagaaagtcaacatcaatattgttggtgactttaaacttaatgaagagatcgccattattttggcatctttttctgcttccacaagtgcttttgtggaaactgtgaaaggtttggattataaagcattcaaacaaattgttgaatcctgtggtaattttaaagttacaaaaggaaaagctaaaaaaggtgcctggaatattggtgaacagaaatcaatactgagtcctctttatgcatttgcatcagaggctgctcgtgttgtacgatcaattttctctcgcactcttgaaactgctcaaaattctgtgcgtgttttacagaaggccgctataacaatactagatggaatttcacagtattcactgagactcattgatgctatgatgttcacatctgatttggctactaacaatctagttgtaatggcctacattacaggtggtgttgttcagttgacttcgcagtggctaactaacatctttggcactgtttatgaaaaactcaaacccgtccttgattggcttgaagagaagtttaaggaaggtgtagagtttcttagagacggttgggaaattgttaaatttatctcaacctgtgcttgtgaaattgtcggtggacaaattgtcacctgtgcaaaggaaattaaggagagtgttcagacattctttaagcttgtaaataaatttttggctttgtgtgctgactctatcattattggtggagctaaacttaaagccttgaatttaggtgaaacatttgtcacgcactcaaagggattgtacagaaagtgtgttaaatccagagaagaaactggcctactcatgcctctaaaagccccaaaagaaattatcttcttagagggagaaacacttcccacagaagtgttaacagaggaagttgtcttgaaaactggtgatttacaaccattagaacaacctactagtgaagctgttgaagctccattggttggtacaccagtttgtattaacgggcttatgttgctcgaaatcaaagacacagaaaagtactgtgcccttgcacctaatatgatggtaacaaacaataccttcacactcaaaggcggtgcaccaacaaaggttacttttggtgatgacactgtgatagaagtgcaaggttacaagagtgtgaatatcacttttgaacttgatgaaaggattgataaagtacttaatgagaagtgctctgcctatacagttgaactcggtacagaagtaaatgagttcgcctgtgttgtggcagatgctgtcataaaaactttgcaaccagtatctgaattacttacaccactgggcattgatttagatgagtggagtatggctacatactacttatttgatgagtctggtgagtttaaattggcttcacatatgtattgttctttctaccctccagatgaggatgaagaagaaggtgattgtgaagaagaagagtttgagccatcaactcaatatgagtatggtactgaagatgattaccaaggtaaacctttggaatttggtgccacttctgctgctcttcaacctgaagaagagcaagaagaagattggttagatgatgatagtcaacaaactgttggtcaacaagacggcagtgaggacaatcagacaactactattcaaacaattgttgaggttcaacctcaattagagatggaacttacaccagttgttcagactattgaagtgaatagttttagtggttatttaaaacttactgacaatgtatacattaaaaatgcagacattgtggaagaagctaaaaaggtaaaaccaacagtggttgttaatgcagccaatgtttaccttaaacatggaggaggtgttgcaggagccttaaataaggctactaacaatgccatgcaagttgaatctgatgattacatagctactaatggaccacttaaagtgggtggtagttgtgttttaagcggacacaatcttgctaaacactgtcttcatgttgtcggcccaaatgttaacaaaggtgaagacattcaacttcttaagagtgcttatgaaaattttaatcagcacgaagttctacttgcaccattattatcagctggtatttttggtgctgaccctatacattctttaagagtttgtgtagatactgttcgcacaaatgtctacttagctgtctttgataaaaatctctatgacaaacttgtttcaagctttttggaaatgaagagtgaaaagcaagttgaacaaaagatcgctgagattcctaaagaggaagttaagccatttataactgaaagtaaaccttcagttgaacagagaaaacaagatgataagaaaatcaaagcttgtgttgaagaagttacaacaactctggaagaaactaagttcctcacagaaaacttgttactttatattgacattaatggcaatcttcatccagattctgccactcttgttagtgacattgacatcactttcttaaagaaagatgctccatatatagtgggtgatgttgttcaagagggtgttttaactgctgtggttatacctactaaaaaggctggtggcactactgaaatgctagcgaaagctttgagaaaagtgccaacagacaattatataaccacttacccgggtcagggtttaaatggttacactgtagaggaggcaaagacagtgcttaaaaagtgtaaaagtgccttttacattctaccatctattatctctaatgagaagcaagaaattcttggaactgtttcttggaatttgcgagaaatgcttgcacatgcagaagaaacacgcaaattaatgcctgtctgtgtggaaactaaagccatagtttcaactatacagcgtaaatataagggtattaaaatacaagagggtgtggttgattatggtgctagattttacttttacaccagtaaaacaactgtagcgtcacttatcaacacacttaacgatctaaatgaaactcttgttacaatgccacttggctatgtaacacatggcttaaatttggaagaagctgctcggtatatgagatctctcaaagtgccagctacagtttctgtttcttcacctgatgctgttacagcgtataatggttatcttacttcttcttctaaaacacctgaagaacattttattgaaaccatctcacttgctggttcctataaagattggtcctattctggacaatctacacaactaggtatagaatttcttaagagaggtgataaaagtgtatattacactagtaatcctaccacattccacctagatggtgaagttatcacctttgacaatcttaagacacttctttctttgagagaagtgaggactattaaggtgtttacaacagtagacaacattaacctccacacgcaagttgtggacatgtcaatgacatatggacaacagtttggtccaacttatttggatggagctgatgttactaaaataaaacctcataattcacatgaaggtaaaacattttatgttttacctaatgatgacactctacgtgttgaggcttttgagtactaccacacaactgatcctagttttctgggtaggtacatgtcagcattaaatcacactaaaaagtggaaatacccacaagttaatggtttaacttctattaaatgggcagataacaactgttatcttgccactgcattgttaacactccaacaaatagagttgaagtttaatccacctgctctacaagatgcttattacagagcaagggctggtgaagctgctaacttttgtgcacttatcttagcctactgtaataagacagtaggtgagttaggtgatgttagagaaacaatgagttacttgtttcaacatgccaatttagattcttgcaaaagagtcttgaacgtggtgtgtaaaacttgtggacaacagcagacaacccttaagggtgtagaagctgttatgtacatgggcacactttcttatgaacaatttaagaaaggtgttcagataccttgtacgtgtggtaaacaagctacaaaatatctagtacaacaggagtcaccttttgttatgatgtcagcaccacctgctcagtatgaacttaagcatggtacatttacttgtgctagtgagtacactggtaattaccagtgtggtcactataaacatataacttctaaagaaactttgtattgcatagacggtgctttacttacaaagtcctcagaatacaaaggtcctattacggatgttttctacaaagaaaacagttacacaacaaccataaaaccagttacttataaattggatggtgttgtttgtacagaaattgaccctaagttggacaattattataagaaagacaattcttatttcacagagcaaccaattgatcttgtaccaaaccaaccatatccaaacgcaagcttcgataattttaagtttgtatgtgataatatcaaatttgctgatgatttaaaccagttaactggttataagaaacctgcttcaagagagcttaaagttacatttttccctgacttaaatggtgatgtggtggctattgattataaacactacacaccctcttttaagaaaggagctaaattgttacataaacctattgtttggcatgttaacaatgcaactaataaagccacgtataaaccaaatacctggtgtatacgttgtctttggagcacaaaaccagttgaaacatcaaattcgtttgatgtactgaagtcagaggacgcgcagggaatggataatcttgcctgcgaagatctaaaaccagtctctgaagaagtagtggaaaatcctaccatacagaaagacgttcttgagtgtaatgtgaaaactaccgaagttgtaggagacattatacttaaaccagcaaataatagtttaaaaattacagaagaggttggccacacagatctaatggctgcttatgtagacaattctagtcttactattaagaaacctaatgaattatctagagtattaggtttgaaaacccttgctactcatggtttagctgctgttaatagtgtcccttgggatactatagctaattatgctaagccttttcttaacaaagttgttagtacaactactaacatagttacacggtgtttaaaccgtgtttgtactaattatatgccttatttctttactttattgctacaattgtgtacttttactagaagtacaaattctagaattaaagcatctatgccgactactatagcaaagaatactgttaagagtgtcggtaaattttgtctagaggcttcatttaattatttgaagtcacctaatttttctaaactgataaatattataatttggtttttactattaagtgtttgcctaggttctttaatctactcaaccgctgctttaggtgttttaatgtctaatttaggcatgccttcttactgtactggttacagagaaggctatttgaactctactaatgtcactattgcaacctactgtactggttctataccttgtagtgtttgtcttagtggtttagattctttagacacctatccttctttagaaactatacaaattaccatttcatcttttaaatgggatttaactgcttttggcttagttgcagagtggtttttggcatatattcttttcactaggtttttctatgtacttggattggctgcaatcatgcaattgtttttcagctattttgcagtacattttattagtaattcttggcttatgtggttaataattaatcttgtacaaatggccccgatttcagctatggttagaatgtacatcttctttgcatcattttattatgtatggaaaagttatgtgcatgttgtagacggttgtaattcatcaacttgtatgatgtgttacaaacgtaatagagcaacaagagtcgaatgtacaactattgttaatggtgttagaaggtccttttatgtctatgctaatggaggtaaaggcttttgcaaactacacaattggaattgtgttaattgtgatacattctgtgctggtagtacatttattagtgatgaagttgcgagagacttgtcactacagtttaaaagaccaataaatcctactgaccagtcttcttacatcgttgatagtgttacagtgaagaatggttccatccatctttactttgataaagctggtcaaaagacttatgaaagacattctctctctcattttgttaacttagacaacctgagagctaataacactaaaggttcattgcctattaatgttatagtttttgatggtaaatcaaaatgtgaagaatcatctgcaaaatcagcgtctgtttactacagtcagcttatgtgtcaacctatactgttactagatcaggcattagtgtctgatgttggtgatagtgcggaagttgcagttaaaatgtttgatgcttacgttaatacgttttcatcaacttttaacgtaccaatggaaaaactcaaaacactagttgcaactgcagaagctgaacttgcaaagaatgtgtccttagacaatgtcttatctacttttatttcagcagctcggcaagggtttgttgattcagatgtagaaactaaagatgttgttgaatgtcttaaattgtcacatcaatctgacatagaagttactggcgatagttgtaataactatatgctcacctataacaaagttgaaaacatgacaccccgtgaccttggtgcttgtattgactgtagtgcgcgtcatattaatgcgcaggtagcaaaaagtcacaacattgctttgatatggaacgttaaagatttcatgtcattgtctgaacaactacgaaaacaaatacgtagtgctgctaaaaagaataacttaccttttaagttgacatgtgcaactactagacaagttgttaatgttgtaacaacaaagatagcacttaagggtggtaaaattgttaataattggttgaagcagttaattaaagttacacttgtgttcctttttgttgctgctattttctatttaataacacctgttcatgtcatgtctaaacatactgacttttcaagtgaaatcataggatacaaggctattgatggtggtgtcactcgtgacatagcatctacagatacttgttttgctaacaaacatgctgattttgacacatggtttagccagcgtggtggtagttatactaatgacaaagcttgcccattgattgctgcagtcataacaagagaagtgggttttgtcgtgcctggtttgcctggcacgatattacgcacaactaatggtgactttttgcatttcttacctagagtttttagtgcagttggtaacatctgttacacaccatcaaaacttatagagtacactgactttgcaacatcagcttgtgttttggctgctgaatgtacaatttttaaagatgcttctggtaagccagtaccatattgttatgataccaatgtactagaaggttctgttgcttatgaaagtttacgccctgacacacgttatgtgctcatggatggctctattattcaatttcctaacacctaccttgaaggttctgttagagtggtaacaacttttgattctgagtactgtaggcacggcacttgtgaaagatcagaagctggtgtttgtgtatctactagtggtagatgggtacttaacaatgattattacagatctttaccaggagttttctgtggtgtagatgctgtaaatttacttactaatatgtttacaccactaattcaacctattggtgctttggacatatcagcatctatagtagctggtggtattgtagctatcgtagtaacatgccttgcctactattttatgaggtttagaagagcttttggtgaatacagtcatgtagttgcctttaatactttactattccttatgtcattcactgtactctgtttaacaccagtttactcattcttacctggtgtttattctgttatttacttgtacttgacattttatcttactaatgatgtttcttttttagcacatattcagtggatggttatgttcacacctttagtacctttctggataacaattgcttatatcatttgtatttccacaaagcatttctattggttctttagtaattacctaaagagacgtgtagtctttaatggtgtttcctttagtacttttgaagaagctgcgctgtgcacctttttgttaaataaagaaatgtatctaaagttgcgtagtgatgtgctattacctcttacgcaatataatagatacttagctctttataataagtacaagtattttagtggagcaatggatacaactagctacagagaagctgcttgttgtcatctcgcaaaggctctcaatgacttcagtaactcaggttctgatgttctttaccaaccaccacaaacctctatcacctcagctgttttgcagagtggttttagaaaaatggcattcccatctggtaaagttgagggttgtatggtacaagtaacttgtggtacaactacacttaacggtctttggcttgatgacgtagtttactgtccaagacatgtgatctgcacctctgaagacatgcttaaccctaattatgaagatttactcattcgtaagtctaatcataatttcttggtacaggctggtaatgttcaactcagggttattggacattctatgcaaaattgtgtacttaagcttaaggttgatacagccaatcctaagacacctaagtataagtttgttcgcattcaaccaggacagactttttcagtgttagcttgttacaatggttcaccatctggtgtttaccaatgtgctatgaggcccaatttcactattaagggttcattccttaatggttcatgtggtagtgttggttttaacatagattatgactgtgtctctttttgttacatgcaccatatggaattaccaactggagttcatgctggcacagacttagaaggtaacttttatggaccttttgttgacaggcaaacagcacaagcagctggtacggacacaactattacagttaatgttttagcttggttgtacgctgctgttataaatggagacaggtggtttctcaatcgatttaccacaactcttaatgactttaaccttgtggctatgaagtacaattatgaacctctaacacaagaccatgttgacatactaggacctctttctgctcaaactggaattgccgttttagatatgtgtgcttcattaaaagaattactgcaaaatggtatgaatggacgtaccatattgggtagtgctttattagaagatgaatttacaccttttgatgttgttagacaatgctcaggtgttactttccaaagtgcagtgaaaagaacaatcaagggtacacaccactggttgttactcacaattttgacttcacttttagttttagtccagagtactcaatggtctttgttcttttttttgtatgaaaatgcctttttaccttttgctatgggtattattgctatgtctgcttttgcaatgatgtttgtcaaacataagcatgcatttctctgtttgtttttgttaccttctcttgccactgtagcttattttaatatggtctatatgcctgctagttgggtgatgcgtattatgacatggttggatatggttgatactagtttgtctggttttaagctaaaagactgtgttatgtatgcatcagctgtagtgttactaatccttatgacagcaagaactgtgtatgatgatggtgctaggagagtgtggacacttatgaatgtcttgacactcgtttataaagtttattatggtaatgctttagatcaagccatttccatgtgggctcttataatctctgttacttctaactactcaggtgtagttacaactgtcatgtttttggccagaggtattgtttttatgtgtgttgagtattgccctattttcttcataactggtaatacacttcagtgtataatgctagtttattgtttcttaggctatttttgtacttgttactttggcctcttttgtttactcaaccgctactttagactgactcttggtgtttatgattacttagtttctacacaggagtttagatatatgaattcacagggactactcccacccaagaatagcatagatgccttcaaactcaacattaaattgttgggtgttggtggcaaaccttgtatcaaagtagccactgtacagtctaaaatgtcagatgtaaagtgcacatcagtagtcttactctcagttttgcaacaactcagagtagaatcatcatctaaattgtgggctcaatgtgtccagttacacaatgacattctcttagctaaagatactactgaagcctttgaaaaaatggtttcactactttctgttttgctttccatgcagggtgctgtagacataaacaagctttgtgaagaaatgctggacaacagggcaaccttacaagctatagcctcagagtttagttcccttccatcatatgcagcttttgctactgctcaagaagcttatgagcaggctgttgctaatggtgattctgaagttgttcttaaaaagttgaagaagtctttgaatgtggctaaatctgaatttgaccgtgatgcagccatgcaacgtaagttggaaaagatggctgatcaagctatgacccaaatgtataaacaggctagatctgaggacaagagggcaaaagttactagtgctatgcagacaatgcttttcactatgcttagaaagttggataatgatgcactcaacaacattatcaacaatgcaagagatggttgtgttcccttgaacataatacctcttacaacagcagccaaactaatggttgtcataccagactataacacatataaaaatacgtgtgatggtacaacatttacttatgcatcagcattgtgggaaatccaacaggttgtagatgcagatagtaaaattgttcaacttagtgaaattagtatggacaattcacctaatttagcatggcctcttattgtaacagctttaagggccaattctgctgtcaaattacagaataatgagcttagtcctgttgcactacgacagatgtcttgtgctgccggtactacacaaactgcttgcactgatgacaatgcgttagcttactacaacacaacaaagggaggtaggtttgtacttgcactgttatccgatttacaggatttgaaatgggctagattccctaagagtgatggaactggtactatctatacagaactggaaccaccttgtaggtttgttacagacacacctaaaggtcctaaagtgaagtatttatactttattaaaggattaaacaacctaaatagaggtatggtacttggtagtttagctgccacagtacgtctacaagctggtaatgcaacagaagtgcctgccaattcaactgtattatctttctgtgcttttgctgtagatgctgctaaagcttacaaagattatctagctagtgggggacaaccaatcactaattgtgttaagatgttgtgtacacacactggtactggtcaggcaataacagttacaccggaagccaatatggatcaagaatcctttggtggtgcatcgtgttgtctgtactgccgttgccacatagatcatccaaatcctaaaggattttgtgacttaaaaggtaagtatgtacaaatacctacaacttgtgctaatgaccctgtgggttttacacttaaaaacacagtctgtaccgtctgcggtatgtggaaaggttatggctgtagttgtgatcaactccgcgaacccatgcttcagtcagctgatgcacaatcgtttttaaacgggtttgcggtgtaagtgcagcccgtcttacaccgtgcggcacaggcactagtactgatgtcgtatacagggcttttgacatctacaatgataaagtagctggttttgctaaattcctaaaaactaattgttgtcgcttccaagaaaaggacgaagatgacaatttaattgattcttactttgtagttaagagacacactttctctaactaccaacatgaagaaacaatttataatttacttaaggattgtccagctgttgctaaacatgacttctttaagtttagaatagacggtgacatggtaccacatatatcacgtcaacgtcttactaaatacacaatggcagacctcgtctatgctttaaggcattttgatgaaggtaattgtgacacattaaaagaaatacttgtcacatacaattgttgtgatgatgattatttcaataaaaaggactggtatgattttgtagaaaacccagatatattacgcgtatacgccaacttaggtgaacgtgtacgccaagctttgttaaaaacagtacaattctgtgatgccatgcgaaatgctggtattgttggtgtactgacattagataatcaagatctcaatggtaactggtatgatttcggtgatttcatacaaaccacgccaggtagtggagttcctgttgtagattcttattattcattgttaatgcctatattaaccttgaccagggctttaactgcagagtcacatgttgacactgacttaacaaagccttacattaagtgggatttgttaaaatatgacttcacggaagagaggttaaaactctttgaccgttattttaaatattgggatcagacataccacccaaattgtgttaactgtttggatgacagatgcattctgcattgtgcaaactttaatgttttattctctacagtgttcccacctacaagttttggaccactagtgagaaaaatatttgttgatggtgttccatttgtagtttcaactggataccacttcagagagctaggtgttgtacataatcaggatgtaaacttacatagctctagacttagttttaaggaattacttgtgtatgctgctgaccctgctatgcacgctgcttctggtaatctattactagataaacgcactacgtgcttttcagtagctgcacttactaacaatgttgcttttcaaactgtcaaacccggtaattttaacaaagacttctatgactttgctgtgtctaagggtttctttaaggaaggaagttctgttgaattaaaacacttcttctttgctcaggatggtaatgctgctatcagcgattatgactactatcgttataatctaccaacaatgtgtgatatcagacaactactatttgtagttgaagttgttgataagtactttgattgttacgatggtggctgtattaatgctaaccaagtcatcgtcaacaacctagacaaatcagctggttttccatttaataaatggggtaaggctagactttattatgattcaatgagttatgaggatcaagatgcacttttcgcatatacaaaacgtaatgtcatccctactataactcaaatgaatcttaagtatgccattagtgcaaagaatagagctcgcaccgtagctggtgtctctatctgtagtactatgaccaatagacagtttcatcaaaaattattgaaatcaatagccgccactagaggagctactgtagtaattggaacaagcaaattctatggtggttggcacaacatgttaaaaactgtttatagtgatgtagaaaaccctcaccttatgggttgggattatcctaaatgtgatagagccatgcctaacatgcttagaattatggcctcacttgttcttgctcgcaaacatacaacgtgttgtagcttgtcacaccgtttctatagattagctaatgagtgtgctcaagtattgagtgaaatggtcatgtgtggcggttcactatatgttaaaccaggtggaacctcatcaggagatgccacaactgcttatgctaatagtgtttttaacatttgtcaagctgtcacggccaatgttaatgcacttttatctactgatggtaacaaaattgccgataagtatgtccgcaatttacaacacagactttatgagtgtctctatagaaatagagatgttgacacagactttgtgaatgagttttacgcatatttgcgtaaacatttctcaatgatgatactctctgacgatgctgttgtgtgtttcaatagcacttatgcatctcaaggtctagtggctagcataaagaactttaagtcagttctttattatcaaaacaatgtttttatgtctgaagcaaaatgttggactgagactgaccttactaaaggacctcatgaattttgctctcaacatacaatgctagttaaacagggtgatgattatgtgtaccttccttacccagatccatcaagaatcctaggggccggctgttttgtagatgatatcgtaaaaacagatggtacacttatgattgaacggttcgtgtctttagctatagatgcttacccacttactaaacatcctaatcaggagtatgctgatgtctttcatttgtacttacaatacataagaaagctacatgatgagttaacaggacacatgttagacatgtattctgttatgcttactaatgataacacttcaaggtattgggaacctgagttttatgaggctatgtacacaccgcatacagtcttacaggctgttggggcttgtgttctttgcaattcacagacttcattaagatgtggtgcttgcatacgtagaccattcttatgttgtaaatgctgttacgaccatgtcatatcaacatcacataaattagtcttgtctgttaatccgtatgtttgcaatgctccaggttgtgatgtcacagatgtgactcaactttacttaggaggtatgagctattattgtaaatcacataaaccacccattagttttccattgtgtgctaatggacaagtttttggtttatataaaaatacatgtgttggtagcgataatgttactgactttaatgcaattgcaacatgtgactggacaaatgctggtgattacattttagctaacacctgtactgaaagactcaagctttttgcagcagaaacgctcaaagctactgaggagacatttaaactgtcttatggtattgctactgtacgtgaagtgctgtctgacagagaattacatctttcatgggaagttggtaaacctagaccaccacttaaccgaaattatgtctttactggttatcgtgtaactaaaaacagtaaagtacaaataggagagtacacctttgaaaaaggtgactatggtgatgctgttgtttaccgaggtacaacaacttacaaattaaatgttggtgattattttgtgctgacatcacatacagtaatgccattaagtgcacctacactagtgccacaagagcactatgttagaattactggcttatacccaacactcaatatctcagatgagttttctagcaatgttgcaaattatcaaaaggttggtatgcaaaagtattctacactccagggaccacctggtactggtaagagtcattttgctattggcctagctctctactacccttctgctcgcatagtgtatacagcttgctctcatgccgctgttgatgcactatgtgagaaggcattaaaatatttgcctatagataaatgtagtagaattatacctgcacgtgctcgtgtagagtgttttgataaattcaaagtgaattcaacattagaacagtatgtcttttgtactgtaaatgcattgcctgagacgacagcagatatagttgtctttgatgaaatttcaatggccacaaattatgatttgagtgttgtcaatgccagattacgtgctaagcactatgtgtacattggcgaccctgctcaattacctgcaccacgcacattgctaactaagggcacactagaaccagaatatttcaattcagtgtgtagacttatgaaaactataggtccagacatgttcctcggaacttgtcggcgttgtcctgctgaaattgttgacactgtgagtgctttggtttatgataataagcttaaagcacataaagacaaatcagctcaatgctttaaaatgttttataagggtgttatcacgcatgatgtttcatctgcaattaacaggccacaaataggcgtggtaagagaattccttacacgtaaccctgcttggagaaaagctgtctttatttcaccttataattcacagaatgctgtagcctcaaagattttgggactaccaactcaaactgttgattcatcacagggctcagaatatgactatgtcatattcactcaaaccactgaaacagctcactcttgtaatgtaaacagatttaatgttgctattaccagagcaaaagtaggcatactttgcataatgtctgatagagacctttatgacaagttgcaatttacaagtcttgaaattccacgtaggaatgtggcaactttacaagctgaaaatgtaacaggactctttaaagattgtagtaaggtaatcactgggttacatcctacacaggcacctacacacctcagtgttgacactaaattcaaaactgaaggtttatgtgttgacatacctggcatacctaaggacatgacctatagaagactcatctctatgatgggttttaaaatgaattatcaagttaatggttaccctaacatgtttatcacccgcgaagaagctataagacatgtacgtgcatggattggcttcgatgtcgaggggtgtcatgctactagagaagctgttggtaccaatttacctttacagctaggtttttctacaggtgttaacctagttgctgtacctacaggttatgttgatacacctaataatacagatttttccagagttagtgctaaaccaccgcctggagatcaatttaaacacctcataccacttatgtacaaaggacttctttggaatgtagtgcgtataaagattgtacaaatgttaagtgacacacttaaaaatctctctgacagagtcgtatttgtcttatgggcacatggctttgagttgacatctatgaagtattttgtgaaaataggacctgagcgcacctgttgtctatgtgatagacgtgccacatgcttttccactgcttcagacacttatgcctgttggcatcattctattggatttgattacgtctataatccgtttatgattgatgttcaacaatggggttttacaggtaacctacaaagcaaccatgatctgtattgtcaagtccatggtaatgcacatgtagctagttgtgatgcaatcatgactaggtgtctagctgtccacgagtgctttgttaagcgtgttgactggactattgaatatcctataattggtgatgaactgaagattaatgcggcttgtagaaaggttcaacacatggttgttaaagctgcattattagcagacaaattcccagttcttcacgacattggtaaccctaaagctattaagtgtgtacctcaagctgatgtagaatggaagttctatgatgcacagccttgtagtgacaaagcttataaaatagaagaattattctattcttatgccacacattctgacaaattcacagatggtgtatgcctattttggaattgcaatgtcgatagatatcctgctaattccattgtttgtagatttgacactagagtgctatctaaccttaacttgcctggttgtgatggtggcagtttgtatgtaaataaacatgcattccacacaccagcttttgataaaagtgcttttgttaatttaaaacaattaccatttttctattactctgacagtccatgtgagtctcatggaaaacaagtagtgtcagatatagattatgtaccactaaagtctgctacgtgtataacacgttgcaatttaggtggtgctgtctgtagacatcatgctaatgagtacagattgtatctcgatgcttataacatgatgatctcagctggctttagcttgtgggtttacaaacaatttgatacttataacctctggaacacttttacaagacttcagagtttagaaaatgtggcttttaatgttgtaaataagggacactttgatggacaacagggtgaagtaccagtttctatcattaataacactgtttacacaaaagttgatggtgttgatgtagaattgtttgaaaataaaacaacattacctgttaatgtagcatttgagctttgggctaagcgcaacattaaaccagtaccagaggtgaaaatactcaataatttgggtgtggacattgctgctaatactgtgatctgggactacaaaagagatgctccagcacatatatctactattggtgtttgttctatgactgacatagccaagaaaccaactgaaacgatttgtgcaccactcactgtcttttttgatggtagagttgatggtcaagtagacttatttagaaatgcccgtaatggtgttcttattacagaaggtagtgttaaaggtttacaaccatctgtaggtcccaaacaagctagtcttaatggagtcacattaattggagaagccgtaaaaacacagttcaattattataagaaagttgatggtgttgtccaacaattacctgaaacttactttactcagagtagaaatttacaagaatttaaacccaggagtcaaatggaaattgatttcttagaattagctatggatgaattcattgaacggtataaattagaaggctatgccttcgaacatatcgtttatggagattttagtcatagtcagttaggtggtttacatctactgattggactagctaaacgttttaaggaatcaccttttgaattagaagattttattcctatggacagtacagttaaaaactatttcataacagatgcgcaaacaggttcatctaagtgtgtgtgttctgttattgatttattacttgatgattttgttgaaataataaaatcccaagatttatctgtagtttctaaggttgtcaaagtgactattgactatacagaaatttcatttatgctttggtgtaaagatggccatgtagaaacattttacccaaaattacaatctagtcaagcgtggcaaccgggtgttgctatgcctaatctttacaaaatgcaaagaatgctattagaaaagtgtgaccttcaaaattatggtgatagtgcaacattacctaaaggcataatgatgaatgtcgcaaaatatactcaactgtgtcaatatttaaacacattaacattagctgtaccctataatatgagagttatacattttggtgctggttctgataaaggagttgcaccaggtacagctgttttaagacagtggttgcctacgggtacgctgcttgtcgattcagatcttaatgactttgtctctgatgcagattcaactttgattggtgattgtgcaactgtacatacagctaataaatgggatctcattattagtgatatgtacgaccctaagactaaaaatgttacaaaagaaaatgactctaaagagggttttttcacttacatttgtgggtttatacaacaaaagctagctcttggaggttccgtggctataaagataacagaacattcttggaatgctgatctttataagctcatgggacacttcgcatggtggacagcctttgttactaatgtgaatgcgtcatcatctgaagcatttttaattggatgtaattatcttggcaaaccacgcgaacaaatagatggttatgtcatgcatgcaaattacatattttggaggaatacaaatccaattcagttgtcttcctattctttatttgacatgagtaaatttccccttaaattaaggggtactgctgttatgtctttaaaagaaggtcaaatcaatgatatgattttatctcttcttagtaaaggtagacttataattagagaaaacaacagagttgttatttctagtgatgttcttgttaacaactaaacgaacaatgtttgtttttcttgttttattgccactagtctctagtcagtgtgttaatcttacaaccagaactcaattaccccctgcatacactaattctttcacacgtggtgtttattaccctgacaaagttttcagatcctcagttttacattcaactcaggacttgttcttacctttcttttccaatgttacttggttccatgctatacatgtctctgggaccaatggtactaagaggtttgataaccctgtcctaccatttaatgatggtgtttattttgcttccactgagaagtctaacataataagaggctggatttttggtactactttagattcgaagacccagtccctacttattgttaataacgctactaatgttgttattaaagtctgtgaatttcaattttgtaatgatccatttttgggtgtttattaccacaaaaacaacaaaagttggatggaaagtgagttcagagtttattctagtgcgaataattgcacttttgaatatgtctctcagccttttcttatggaccttgaaggaaaacagggtaatttcaaaaatcttagggaatttgtgtttaagaatattgatggttattttaaaatatattctaagcacacgcctattaatttagtgcgtgatctccctcagggtttttcggctttagaaccattggtagatttgccaataggtattaacatcactaggtttcaaactttacttgctttacatagaagttatttgactcctggtgattcttcttcaggttggacagctggtgctgcagcttattatgtgggttatcttcaacctaggacttttctattaaaatataatgaaaatggaaccattacagatgctgtagactgtgcacttgaccctctctcagaaacaaagtgtacgttgaaatccttcactgtagaaaaaggaatctatcaaacttctaactttagagtccaaccaacagaatctattgttagatttcctaatattacaaacttgtgcccttttggtgaagtttttaacgccaccagatttgcatctgtttatgcttggaacaggaagagaatcagcaactgtgttgctgattattctgtcctatataattccgcatcattttccacttttaagtgttatggagtgtctcctactaaattaaatgatctctgctttactaatgtctatgcagattcatttgtaattagaggtgatgaagtcagacaaatcgctccagggcaaactggaaagattgctgattataattataaattaccagatgattttacaggctgcgttatagcttggaattctaacaatcttgattctaaggttggtggtaattataattacctgtatagattgtttaggaagtctaatctcaaaccttttgagagagatatttcaactgaaatctatcaggccggtagcacaccttgtaatggtgttgaaggttttaattgttactttcctttacaatcatatggtttccaacccactaatggtgttggttaccaaccatacagagtagtagtactttcttttgaacttctacatgcaccagcaactgtttgtggacctaaaaagtctactaatttggttaaaaacaaatgtgtcaatttcaacttcaatggtttaacaggcacaggtgttcttactgagtctaacaaaaagtttctgcctttccaacaatttggcagagacattgctgacactactgatgctgtccgtgatccacagacacttgagattcttgacattacaccatgttcttttggtggtgtcagtgttataacaccaggaacaaatacttctaaccaggttgctgttctttatcaggatgttaactgcacagaagtccctgttgctattcatgcagatcaacttactcctacttggcgtgtttattctacaggttctaatgtttttcaaacacgtgcaggctgtttaataggggctgaacatgtcaacaactcatatgagtgtgacatacccattggtgcaggtatatgcgctagttatcagactcagactaattctcctcggcgggcacgtagtgtagctagtcaatccatcattgcctacactatgtcacttggtgcagaaaattcagttgcttactctaataactctattgccatacccacaaattttactattagtgttaccacagaaattctaccagtgtctatgaccaagacatcagtagattgtacaatgtacatttgtggtgattcaactgaatgcagcaatcttttgttgcaatatggcagtttttgtacacaattaaaccgtgctttaactggaatagctgttgaacaagacaaaaacacccaagaagtttttgcacaagtcaaacaaatttacaaaacaccaccaattaaagattttggtggttttaatttttcacaaatattaccagatccatcaaaaccaagcaagaggtcatttattgaagatctacttttcaacaaagtgacacttgcagatgctggcttcatcaaacaatatggtgattgccttggtgatattgctgctagagacctcatttgtgcacaaaagtttaacggccttactgttttgccacctttgctcacagatgaaatgattgctcaatacacttctgcactgttagcgggtacaatcacttctggttggacctttggtgcaggtgctgcattacaaataccatttgctatgcaaatggcttataggtttaatggtattggagttacacagaatgttctctatgagaaccaaaaattgattgccaaccaatttaatagtgctattggcaaaattcaagactcactttcttccacagcaagtgcacttggaaaacttcaagatgtggtcaaccaaaatgcacaagctttaaacacgcttgttaaacaacttagctccaattttggtgcaatttcaagtgttttaaatgatatcctttcacgtcttgacaaagttgaggctgaagtgcaaattgataggttgatcacaggcagacttcaaagtttgcagacatatgtgactcaacaattaattagagctgcagaaatcagagcttctgctaatcttgctgctactaaaatgtcagagtgtgtacttggacaatcaaaaagagttgatttttgtggaaagggctatcatcttatgtccttccctcagtcagcacctcatggtgtagtcttcttgcatgtgacttatgtccctgcacaagaaaagaacttcacaactgctcctgccatttgtcatgatggaaaagcacactttcctcgtgaaggtgtctttgtttcaaatggcacacactggtttgtaacacaaaggaatttttatgaaccacaaatcattactacagacaacacatttgtgtctggtaactgtgatgttgtaataggaattgtcaacaacacagtttatgatcctttgcaacctgaattagactcattcaaggaggagttagataaatattttaagaatcatacatcaccagatgttgatttaggtgacatctctggcattaatgcttcagttgtaaacattcaaaaagaaattgaccgcctcaatgaggttgccaagaatttaaatgaatctctcatcgatctccaagaacttggaaagtatgagcagtatataaaatggccatggtacatttggctaggttttatagctggcttgattgccatagtaatggtgacaattatgctttgctgtatgaccagttgctgtagttgtctcaagggctgttgttcttgtggatcctgctgcaaatttgatgaagacgactctgagccagtgctcaaaggagtcaaattacattacacataaacgaacttatggatttgtttatgagaatcttcacaattggaactgtaactttgaagcaaggtgaaatcaaggatgctactccttcagattttgttcgcgctactgcaacgataccgatacaagcctcactccctttcggatggcttattgttggcgttgcacttcttgctgtttttcagagcgcttccaaaatcataaccctcaaaaagagatggcaactagcactctccaagggtgttcactttgtttgcaacttgctgttgttgtttgtaacagtttactcacaccttttgctcgttgctgctggccttgaagccccttttctctatctttatgctttagtctacttcttgcagagtataaactttgtaagaataataatgaggctttggctttgctggaaatgccgttccaaaaacccattactttatgatgccaactattttctttgctggcatactaattgttacgactattgtataccttacaatagtgtaacttcttcaattgtcattacttcaggtgatggcacaacaagtcctatttctgaacatgactaccagattggtggttatactgaaaaatgggaatctggagtaaaagactgtgttgtattacacagttacttcacttcagactattaccagctgtactcaactcaattgagtacagacactggtgttgaacatgttaccttcttcatctacaataaaattgttgatgagcctgaagaacatgtccaaattcacacaatcgacggttcatccggagttgttaatccagtaatggaaccaatttatgatgaaccgacgacgactactagcgtgcctttgtaagcacaagctgatgagtacgaacttatgtactcattcgtttcggaagagacaggtacgttaatagttaatagcgtacttctttttcttgctttcgtggtattcttgctagttacactagccatccttactgcgcttcgattgtgtgcgtactgctgcaatattgttaacgtgagtcttgtaaaaccttctttttacgtttactctcgtgttaaaaatctgaattcttctagagttcctgatcttctggtctaaacgaactaaatattatattagtttttctgtttggaactttaattttagccatggcagattccaacggtactattaccgttgaagagcttaaaaagctccttgaacaatggaacctagtaataggtttcctattccttacatggatttgtcttctacaatttgcctatgccaacaggaataggtttttgtatataattaagttaattttcctctggctgttatggccagtaactttagcttgttttgtgcttgctgctgtttacagaataaattggatcaccggtggaattgctatcgcaatggcttgtcttgtaggcttgatgtggctcagctacttcattgcttctttcagactgtttgcgcgtacgcgttccatgtggtcattcaatccagaaactaacattcttctcaacgtgccactccatggcactattctgaccagaccgcttctagaaagtgaactcgtaatcggagctgtgatccttcgtggacatcttcgtattgctggacaccatctaggacgctgtgacatcaaggacctgcctaaagaaatcactgttgctacatcacgaacgctttcttattacaaattgggagcttcgcagcgtgtagcaggtgactcaggttttgctgcatacagtcgctacaggattggcaactataaattaaacacagaccattccagtagcagtgacaatattgctttgcttgtacagtaagtgacaacagatgtttcatctcgttgactttcaggttactatagcagagatattactaattattatgaggacttttaaagtttccatttggaatcttgattacatcataaacctcataattaaaaatttatctaagtcactaactgagaataaatattctcaattagatgaagagcaaccaatggagattgattaaacgaacatgaaaattattcttttcttggcactgataacactcgctacttgtgagctttatcactaccaagagtgtgttagaggtacaacagtacttttaaaagaaccttgctcttctggaacatacgagggcaattcaccatttcatcctctagctgataacaaatttgcactgacttgctttagcactcaatttgcttttgcttgtcctgacggcgtaaaacacgtctatcagttacgtgccagatcagtttcacctaaactgttcatcagacaagaggaagttcaagaactttactctccaatttttcttattgttgcggcaatagtgtttataacactttgcttcacactcaaaagaaagacagaatgattgaactttcattaattgacttctatttgtgctttttagcctttctgctattccttgttttaattatgcttattatcttttggttctcacttgaactgcaagatcataatgaaacttgtcacgcctaaacgaacatgaaatttcttgttttcttaggaatcatcacaactgtagctgcatttcaccaagaatgtagtttacagtcatgtactcaacatcaaccatatgtagttgatgacccgtgtcctattcacttctattctaaatggtatattagagtaggagctagaaaatcagcacctttaattgaattgtgcgtggatgaggctggttctaaatcacccattcagtacatcgatatcggtaattatacagtttcctgtttaccttttacaattaattgccaggaacctaaattgggtagtcttgtagtgcgttgttcgttctatgaagactttttagagtatcatgacgttcgtgttgttttagatttcatctaaacgaacaaactaaaatgtctgataatggaccccaaaatcagcgaaatgcaccccgcattacgtttggtggaccctcagattcaactggcagtaaccagaatggagaacgcagtggggcgcgatcaaaacaacgtcggccccaaggtttacccaataatactgcgtcttggttcaccgctctcactcaacatggcaaggaagaccttaaattccctcgaggacaaggcgttccaattaacaccaatagcagtccagatgaccaaattggctactaccgaagagctaccagacgaattcgtggtggtgacggtaaaatgaaagatctcagtccaagatggtatttctactacctaggaactgggccagaagctggacttccctatggtgctaacaaagacggcatcatatgggttgcaactgagggagccttgaatacaccaaaagatcacattggcacccgcaatcctgctaacaatgctgcaatcgtgctacaacttcctcaaggaacaacattgccaaaaggcttctacgcagaagggagcagaggcggcagtcaagcctcttctcgttcctcatcacgtagtcgcaacagttcaagaaattcaactccaggcagcagtaggggaacttctcctgctagaatggctggcaatggcggtgatgctgctcttgctttgctgctgcttgacagattgaaccagcttgagagcaaaatgtctggtaaaggccaacaacaacaaggccaaactgtcactaagaaatctgctgctgaggcttctaagaagcctcggcaaaaacgtactgccactaaagcatacaatgtaacacaagctttcggcagacgtggtccagaacaaacccaaggaaattttggggaccaggaactaatcagacaaggaactgattacaaacattggccgcaaattgcacaatttgcccccagcgcttcagcgttcttcggaatgtcgcgcattggcatggaagtcacaccttcgggaacgtggttgacctacacaggtgccatcaaattggatgacaaagatccaaatttcaaagatcaagtcattttgctgaataagcatattgacgcatacaaaacattcccaccaacagagcctaaaaaggacaaaaagaagaaggctgatgaaactcaagccttaccgcagagacagaagaaacagcaaactgtgactcttcttcctgctgcagatttggatgatttctccaaacaattgcaacaatccatgagcagtgctgactcaactcaggcctaaactcatgcagaccacacaaggcagatgggctatataaacgttttcgcttttccgtttacgatatatagtctactcttgtgcagaatgaattctcgtaactacatagcacaagtagatgtagttaactttaatctcacatagcaatctttaatcagtgtgtaacattagggaggacttgaaagagccaccacattttcaccgaggccacgcggagtacgatcgagtgtacagtgaacaatgctagggagagctgcctatatggaagagccctaatgtgtaaaattaattttagtagtgctatccccatgtgattttaatagcttcttaggagaatgacaaaaa

SEQ ID NO: 10 - DNA, 3903 bp, Artificial
  Synthetic DNA
gaattcggcttataatgtagctccttcatcaatcatacattttttcaccattacttcttccatgtccaatatgatcatgtgagaatactaaaattcctaacgatgatatgttttcagctagttcgtcataacgtccagaatgtttaccagctccatgacttatgaatactaatgccttaggatatgtaataggtttccaatatttacaatatatgtaatcattgtccagattgaacatacagtttgcactcatgattcacgttatataactatcaatattaacagttcgtttgatgatcatattatttttatgttttattgataattgtaaaaacatacaattaaatcaatatagaggaaggagacggctactgtcttttgtgagatagtcatggcgactaaattagattatgaggatgctgttttttactttgtggatgatgataaaatatgtagtcgcgactccatcatcgatctaataaatgaatatattacgtggagaaatcatgttatagtgtttaacaaagatattaccagttgtggaagactgtacaaggaattgatgaagttcgatgatgtcgctatacggtactatggtattgataaaattaatgagattgtcgaagctatgagcgaaggagaccactacatcaattttacaaaagtccatgatcaggaaagtttattcgctaccataggaatatgtgctaaaatcactgaacattggggatacaaaaagatttcagaatctagattccaatcattgggaaacattacagatctgatgaccgacgataatataaacatcttgatactttttctagaaaaaaaattgaattgatgatataggggtcttcataacgcataattattacgttagcattctatatccgtgttaaaaaaaattatcctatcatgtatttgagagttttatatgtagcaaacatgatagctgtgatgccaataagctttagatattcacgcggcatgcctgcaggtcgacgtttaaacgcgatcgccgcgtgctagtgttagggatggtattatctggtggtgaaatgtccgttatataatctacaaaacaatcatcgcatatagtatgcgatagtagagtaaacatttttatagtttttactggattcatacatcgtctacccaattcggttataaatgaaattgtcgccaatcttacacccaaccccttgttatccattagtatagtattaacttcgttatttatgtcataaactgtaaatgattttgtagatgccatatcatacatgatattcatgtccctattataatcattactaactttatcacaatatatgttgataatatctatatatgatctagtctttgtgggcaactgtctatacaagtcgtctaaacgttgtttactcatatagtatcgaacagccatcattacatggtcccgttccgttgatagataatcgagtatgttagtggacttgtcaaatctatataccatattttctggaagtggatatacatagtcgtgatcaacattattgctagcctcatcttctatatcctgtactataccattatctatatcctctatatcctgtactataccattatctatatcctctatatcatctacataatctacgatattattacacataaacatcgacaacatactattgtttattatctaagtcctgttgatccaaacccttgatctcctctatctgtactatctagagattgtacttcttccagttctggataatatatacgttgatagattagctgagctattctatctccagtatttacattaaacgtacattttccattattaataagaatgactcctatgtttcccctataatcttcgtctattacaccacctcctaagccgaattctctagatatcgctcaatactgaccatttaaatcatacctgacctccatagcagaaagtcaaaagcctccgaccggaggcttttgacttgatcggcacgtaagaggttccaactttcaccataatgaaataagatcactaccgggcgtattttttgagttatcgagattttcaggagctaaggaagctaaaatgagtattcaacatttccgtgtcgcccttattcccttttttgcggcattttgccttcctgtttttgctcacccagaaacgctggtgaaagtaaaagatgctgaagatcagttgggtgcacgagtgggttacatcgaactggatctcaacagcggtaagatccttgagagtttacgccccgaagaacgttttccaatgatgagcacttttaaagttctgctatgtggcgcggtattatcccgtattgacgccgggcaagagcaactcggtcgccgcatacactattctcagaatgacttggttgagtactcaccagtcacagaaaagcatctcacggatggcatgacagtaagagaattatgcagtgctgccataaccatgagtgataacactgcggccaacttacttctggcaacgatcggaggaccgaaggagctaaccgcttttttgcacaacatgggggatcatgtaactcgccttgatcgttgggaaccggagctgaatgaagccataccaaacgacgagcgtgacaccacgatgcctgtagcaatggcaacaacgttgcgcaaactattaactggcgaactacttactctagcttcccggcaacaattaatagactggatggaggcggataaagttgcaggatcacttctgcgctcggccctcccggctggctggtttattgctgataaatctggagccggtgagcgtgggtctcgcggtatcattgcagcactggggccagatggtaagccctcccgcatcgtagttatctacacgacggggagtcaggcaactatggatgaacgaaatagacagatcgctgagataggtgcctcactgattaagcattggtaagtgaccaaacaggaaaaaaccgcccttaacatggcccgctttatcagaagccagacattaacgcttctggagaaactcaacgagctggacgcggatgaacaggcagacatctgtgaatcgcttcacgaccacgctgatgagctttaccgcagctgcctcgcgcgtttcggtgatgacggtgaaaacctctgatgagggcccaaatgtaatcacctggctcaccttcgggtgggcctttctgcgttgctggcgtttttccataggctccgcccccctgacgagcatcacaaaaatcgatgctcaagtcagaggtggcgaaacccgacaggactataaagataccaggcgtttccccctggaagctccctcgtgcgctctcctgttccgaccctgccgcttaccggatacctgtccgcctttctcccttcgggaagcgtggcgctttctcatagctcacgctgtaggtatctcagttcggtgtaggtcgttcgctccaagctgggctgtgtgcacgaaccccccgttcagcccgaccgctgcgccttatccggtaactatcgtcttgagtccaacccggtaagacacgacttatcgccactggcagcagccactggtaacaggattagcagagcgaggtatgtaggcggtgctacagagttcttgaagtggtggcctaactacggctacactagaagaacagtatttggtatctgcgctctgctgaagccagttacctcggaaaaagagttggtagctcttgatccggcaaacaaaccaccgctggtagcggtggtttttttgtttgcaagcagcagattacgcgcagaaaaaaaggatctcaagaagatcctttgattttctaccgaagaaaggcccacccgtgaaggtgagccagtgagttgattgcagtccagttacgctggagtctgaggctcgtcctgaatgatatcaagctt

SEQ ID NO: 11 - DNA, 20 bp, Artificial
  Synthetic DNA
tggggytttacrggtaacct

SEQ ID NO: 12 - DNA, 21 bp, Artificial
  Synthetic DNA
aacrcgcttaacaaagcactc

SEQ ID NO: 13 - DNA, 24 bp, Artificial
  Synthetic DNA
tagttgtgatgcwatcatgactag